European Patent Specification EP 3 434 776 B1, published September 2, 2026. Title: METHODS, MODELS, SYSTEMS, AND APPARATUS FOR IDENTIFYING TARGET SEQUENCES FOR CAS ENZYMES OR CRISPR-CAS SYSTEMS FOR TARGET SEQUENCES AND CONVEYING RESULTS THEREOF. Applicant: THE BROAD INSTITUTE, INC. Application PCT/US2013/074812. The sequence listing filed with the application follows.

SEQUENCE LISTING (1076 sequences)

SEQ ID NO: 1 - RNA, 12 nt, Artificial Sequence
  source: /note="Description of Artificial Sequence: Synthetic oligonucleotide"
guuuuagagcua

SEQ ID NO: 2 - protein, 7 aa, Simian virus 40
PKKKRKV

SEQ ID NO: 3 - protein, 16 aa, Unknown
  source: /note="Description of Unknown: Nucleoplasmin bipartite NLS sequence"
KRPAATKKAGQAKKKK

SEQ ID NO: 4 - protein, 9 aa, Unknown
  source: /note="Description of Unknown: C-myc NLS sequence"
PAAKRVKLD

SEQ ID NO: 5 - protein, 11 aa, Unknown
  source: /note="Description of Unknown: C-myc NLS sequence"
RQRRNELKRSP

SEQ ID NO: 6 - protein, 38 aa, Homo sapiens
NQSSNFGPMKGGNFGGRSSGPYGGGGQYFAKPRNQGGY

SEQ ID NO: 7 - protein, 42 aa, Unknown
  source: /note="Description of Unknown: IBB domain from importin-alpha sequence"
RMRIZFKNKGKDTAELRRRRVEVSVELRKAKKDEQILKRRNV

SEQ ID NO: 8 - protein, 8 aa, Unknown
  source: /note="Description of Unknown: Myoma T protein sequence"
VSRKRPRP

SEQ ID NO: 9 - protein, 8 aa, Unknown
  source: /note="Description of Unknown: Myoma T protein sequence"
PPKKARED

SEQ ID NO: 10 - protein, 8 aa, Homo sapiens
PQPKKKPL

SEQ ID NO: 11 - protein, 12 aa, Mus musculus
SALIKKKKKMAP

SEQ ID NO: 12 - protein, 5 aa, Influenza virus
DRLRR

SEQ ID NO: 13 - protein, 7 aa, Influenza virus
PKQKKRK

SEQ ID NO: 14 - protein, 10 aa, Hepatitus delta virus
RKLKKKIKKL

SEQ ID NO: 15 - protein, 10 aa, Mus musculus
REKKKFLKRR

SEQ ID NO: 16 - protein, 20 aa, Homo sapiens
KRKGDEVDGVDEVAKKKSKK

SEQ ID NO: 17 - protein, 17 aa, Homo sapiens
RKCLQAGMNLEARKTKK

SEQ ID NO: 18 - DNA, 27 bp, Artificial Sequence
  source: /note="Description of Artificial Sequence: Synthetic oligonucleotide"
  modified_base (1)..(20): a, c, t or g
  modified_base (21)..(22): a, c, t, g, unknown or other
nnnnnnnnnnnnnnnnnnnnnnagaaw

SEQ ID NO: 19 - DNA, 19 bp, Artificial Sequence
  source: /note="Description of Artificial Sequence: Synthetic oligonucleotide"
  modified_base (1)..(12): a, c, t or g
  modified_base (13)..(14): a, c, t, g, unknown or other
nnnnnnnnnnnnnnagaaw

SEQ ID NO: 20 - DNA, 27 bp, Artificial Sequence
  source: /note="Description of Artificial Sequence: Synthetic oligonucleotide"
  modified_base (1)..(20): a, c, t or g
  modified_base (21)..(22): a, c, t, g, unknown or other
nnnnnnnnnnnnnnnnnnnnnnagaaw

SEQ ID NO: 21 - DNA, 18 bp, Artificial Sequence
  source: /note="Description of Artificial Sequence: Synthetic oligonucleotide"
  modified_base (1)..(11): a, c, t or g
  modified_base (12)..(13): a, c, t, g, unknown or other
nnnnnnnnnnnnnagaaw

SEQ ID NO: 22 - DNA, 137 bp, Artificial Sequence
  source: /note="Description of Artificial Sequence: Synthetic polynucleotide"
  modified_base (1)..(20): a, c, t, g, unknown or other
nnnnnnnnnnnnnnnnnnnngtttttgtactctcaagatttagaaataaatcttgcagaagctacaaagataaggcttcatgccgaaatcaacaccctgtcattttatggcagggtgttttcgttatttaatttttt

SEQ ID NO: 23 - DNA, 123 bp, Artificial Sequence
  source: /note="Description of Artificial Sequence: Synthetic polynucleotide"
  modified_base (1)..(20): a, c, t, g, unknown or other
nnnnnnnnnnnnnnnnnnnngtttttgtactctcagaaatgcagaagctacaaagataaggcttcatgccgaaatcaacaccctgtcattttatggcagggtgttttcgttatttaatttttt

SEQ ID NO: 24 - DNA, 110 bp, Artificial Sequence
  source: /note="Description of Artificial Sequence: Synthetic polynucleotide"
  modified_base (1)..(20): a, c, t, g, unknown or other
nnnnnnnnnnnnnnnnnnnngtttttgtactctcagaaatgcagaagctacaaagataaggcttcatgccgaaatcaacaccctgtcattttatggcagggtgttttttt

SEQ ID NO: 25 - DNA, 102 bp, Artificial Sequence
  source: /note="Description of Artificial Sequence: Synthetic polynucleotide"
  modified_base (1)..(20): a, c, t, g, unknown or other
nnnnnnnnnnnnnnnnnnnngttttagagctagaaatagcaagttaaaataaggctagtccgttatcaacttgaaaaagtggcaccgagtcggtgctttttt

SEQ ID NO: 26 - DNA, 88 bp, Artificial Sequence
  source: /note="Description of Artificial Sequence: Synthetic oligonucleotide"
  modified_base (1)..(20): a, c, t, g, unknown or other
nnnnnnnnnnnnnnnnnnnngttttagagctagaaatagcaagttaaaataaggctagtccgttatcaacttgaaaaagtgttttttt

SEQ ID NO: 27 - DNA, 76 bp, Artificial Sequence
  source: /note="Description of Artificial Sequence: Synthetic oligonucleotide"
  modified_base (1)..(20): a, c, t, g, unknown or other
nnnnnnnnnnnnnnnnnnnngttttagagctagaaatagcaagttaaaataaggctagtccgttatcatttttttt

SEQ ID NO: 28 - DNA, 22 bp, Homo sapiens
  modified_base (20)..(20): a, c, t, g, unknown or other
aggccccagtggctgctctnaa

SEQ ID NO: 29 - DNA, 22 bp, Homo sapiens
  modified_base (20)..(20): a, c, t, g, unknown or other
acatcaaccggtggcgcatnat

SEQ ID NO: 30 - DNA, 22 bp, Homo sapiens
  modified_base (20)..(20): a, c, t, g, unknown or other
aaggtgtggttccagaaccnac

SEQ ID NO: 31 - DNA, 22 bp, Homo sapiens
  modified_base (20)..(20): a, c, t, g, unknown or other
ccatcacatcaaccggtggnag

SEQ ID NO: 32 - DNA, 22 bp, Homo sapiens
  modified_base (20)..(20): a, c, t, g, unknown or other
aaacggcagaagctggaggnta

SEQ ID NO: 33 - DNA, 22 bp, Homo sapiens
  modified_base (20)..(20): a, c, t, g, unknown or other
ggcagaagctggaggaggantt

SEQ ID NO: 34 - DNA, 22 bp, Homo sapiens
  modified_base (20)..(20): a, c, t, g, unknown or other
ggtgtggttccagaaccggntc

SEQ ID NO: 35 - DNA, 22 bp, Homo sapiens
  modified_base (20)..(20): a, c, t, g, unknown or other
aaccggaggacaaagtacantg

SEQ ID NO: 36 - DNA, 22 bp, Homo sapiens
  modified_base (20)..(20): a, c, t, g, unknown or other
ttccagaaccggaggacaanca

SEQ ID NO: 37 - DNA, 22 bp, Homo sapiens
  modified_base (20)..(20): a, c, t, g, unknown or other
gtgtggttccagaaccgganct

SEQ ID NO: 38 - DNA, 22 bp, Homo sapiens
  modified_base (20)..(20): a, c, t, g, unknown or other
tccagaaccggaggacaaancc

SEQ ID NO: 39 - DNA, 22 bp, Homo sapiens
  modified_base (20)..(20): a, c, t, g, unknown or other
cagaagctggaggaggaagncg

SEQ ID NO: 40 - DNA, 22 bp, Homo sapiens
  modified_base (20)..(20): a, c, t, g, unknown or other
catcaaccggtggcgcattnga

SEQ ID NO: 41 - DNA, 22 bp, Homo sapiens
  modified_base (20)..(20): a, c, t, g, unknown or other
gcagaagctggaggaggaangt

SEQ ID NO: 42 - DNA, 22 bp, Homo sapiens
  modified_base (20)..(20): a, c, t, g, unknown or other
cctccctccctggcccaggngc

SEQ ID NO: 43 - DNA, 22 bp, Homo sapiens
  modified_base (20)..(20): a, c, t, g, unknown or other
tcatctgtgcccctccctcnaa

SEQ ID NO: 44 - DNA, 22 bp, Homo sapiens
  modified_base (20)..(20): a, c, t, g, unknown or other
gggaggacatcgatgtcacnat

SEQ ID NO: 45 - DNA, 22 bp, Homo sapiens
  modified_base (20)..(20): a, c, t, g, unknown or other
caaacggcagaagctggagnac

SEQ ID NO: 46 - DNA, 22 bp, Homo sapiens
  modified_base (20)..(20): a, c, t, g, unknown or other
gggtgggcaaccacaaaccnag

SEQ ID NO: 47 - DNA, 22 bp, Homo sapiens
  modified_base (20)..(20): a, c, t, g, unknown or other
ggtgggcaaccacaaacccnta

SEQ ID NO: 48 - DNA, 22 bp, Homo sapiens
  modified_base (20)..(20): a, c, t, g, unknown or other
ggctcccatcacatcaaccntt

SEQ ID NO: 49 - DNA, 22 bp, Homo sapiens
  modified_base (20)..(20): a, c, t, g, unknown or other
gaagggcctgagtccgagcntc

SEQ ID NO: 50 - DNA, 22 bp, Homo sapiens
  modified_base (20)..(20): a, c, t, g, unknown or other
caaccggtggcgcattgccntg

SEQ ID NO: 51 - DNA, 22 bp, Homo sapiens
  modified_base (20)..(20): a, c, t, g, unknown or other
aggaggaagggcctgagtcnca

SEQ ID NO: 52 - DNA, 22 bp, Homo sapiens
  modified_base (20)..(20): a, c, t, g, unknown or other
agctggaggaggaagggccnct

SEQ ID NO: 53 - DNA, 22 bp, Homo sapiens
  modified_base (20)..(20): a, c, t, g, unknown or other
gcattgccacgaagcaggcncc

SEQ ID NO: 54 - DNA, 22 bp, Homo sapiens
  modified_base (20)..(20): a, c, t, g, unknown or other
attgccacgaagcaggccancg

SEQ ID NO: 55 - DNA, 22 bp, Homo sapiens
  modified_base (20)..(20): a, c, t, g, unknown or other
agaaccggaggacaaagtanga

SEQ ID NO: 56 - DNA, 22 bp, Homo sapiens
  modified_base (20)..(20): a, c, t, g, unknown or other
tcaaccggtggcgcattgcngt

SEQ ID NO: 57 - DNA, 22 bp, Homo sapiens
  modified_base (20)..(20): a, c, t, g, unknown or other
gaagctggaggaggaagggngc

SEQ ID NO: 58 - DNA, 23 bp, Artificial Sequence
  source: /note="Description of Artificial Sequence: Synthetic oligonucleotide"
gccaaattggacgaccctcgcgg

SEQ ID NO: 59 - DNA, 23 bp, Artificial Sequence
  source: /note="Description of Artificial Sequence: Synthetic oligonucleotide"
cgaggagacccccgtttcggtgg

SEQ ID NO: 60 - DNA, 23 bp, Artificial Sequence
  source: /note="Description of Artificial Sequence: Synthetic oligonucleotide"
cccgccgccgccgtggctcgagg

SEQ ID NO: 61 - DNA, 23 bp, Artificial Sequence
  source: /note="Description of Artificial Sequence: Synthetic oligonucleotide"
tgagctctacgagatccacaagg

SEQ ID NO: 62 - DNA, 23 bp, Artificial Sequence
  source: /note="Description of Artificial Sequence: Synthetic oligonucleotide"
ctcaaaattcataccggttgtgg

SEQ ID NO: 63 - DNA, 23 bp, Artificial Sequence
  source: /note="Description of Artificial Sequence: Synthetic oligonucleotide"
cgttaaacaacaaccggacttgg

SEQ ID NO: 64 - DNA, 23 bp, Artificial Sequence
  source: /note="Description of Artificial Sequence: Synthetic oligonucleotide"
ttcaccccgcggcgctgaatggg

SEQ ID NO: 65 - DNA, 23 bp, Artificial Sequence
  source: /note="Description of Artificial Sequence: Synthetic oligonucleotide"
accactaccagtccgtccacagg

SEQ ID NO: 66 - DNA, 23 bp, Artificial Sequence
  source: /note="Description of Artificial Sequence: Synthetic oligonucleotide"
cactgcttaagcctcgctcgagg

SEQ ID NO: 67 - DNA, 23 bp, Artificial Sequence
  source: /note="Description of Artificial Sequence: Synthetic oligonucleotide"
tcaccagcaatattcgctcgagg

SEQ ID NO: 68 - DNA, 23 bp, Artificial Sequence
  source: /note="Description of Artificial Sequence: Synthetic oligonucleotide"
caccagcaatattccgctcgagg

SEQ ID NO: 69 - DNA, 23 bp, Artificial Sequence
  source: /note="Description of Artificial Sequence: Synthetic oligonucleotide"
tagcaacagacatacgctcgagg

SEQ ID NO: 70 - DNA, 23 bp, Artificial Sequence
  source: /note="Description of Artificial Sequence: Synthetic oligonucleotide"
gggcagtagtaatacgctcgagg

SEQ ID NO: 71 - DNA, 23 bp, Artificial Sequence
  source: /note="Description of Artificial Sequence: Synthetic oligonucleotide"
ccaattcccatacattattgtac

SEQ ID NO: 72 - DNA, 33 bp, Homo sapiens
ggacatcgatgtcacctccaatgactagggtgg

SEQ ID NO: 73 - DNA, 33 bp, Homo sapiens
cattggaggtgacatcgatgtcctccccattgg

SEQ ID NO: 74 - DNA, 33 bp, Homo sapiens
ggaagggcctgagtccgagcagaagaagaaggg

SEQ ID NO: 75 - DNA, 33 bp, Homo sapiens
ggtggcgagaggggccgagattgggtgttcagg

SEQ ID NO: 76 - DNA, 33 bp, Homo sapiens
atgcaggagggtggcgagaggggccgagattgg

SEQ ID NO: 77 - DNA, 23 bp, Homo sapiens
gtcacctccaatgactagggtgg

SEQ ID NO: 78 - DNA, 23 bp, Homo sapiens
gacatcgatgtcctccccattgg

SEQ ID NO: 79 - DNA, 23 bp, Homo sapiens
gagtccgagcagaagaagaaggg

SEQ ID NO: 80 - DNA, 23 bp, Homo sapiens
gcgccaccggttgatgtgatggg

SEQ ID NO: 81 - DNA, 23 bp, Homo sapiens
ggggcacagatgagaaactcagg

SEQ ID NO: 82 - DNA, 23 bp, Homo sapiens
gtacaaacggcagaagctggagg

SEQ ID NO: 83 - DNA, 23 bp, Homo sapiens
ggcagaagctggaggaggaaggg

SEQ ID NO: 84 - DNA, 23 bp, Homo sapiens
ggagcccttcttcttctgctcgg

SEQ ID NO: 85 - DNA, 23 bp, Homo sapiens
gggcaaccacaaacccacgaggg

SEQ ID NO: 86 - DNA, 23 bp, Homo sapiens
gctcccatcacatcaaccggtgg

SEQ ID NO: 87 - DNA, 23 bp, Homo sapiens
gtggcgcattgccacgaagcagg

SEQ ID NO: 88 - DNA, 23 bp, Homo sapiens
ggcagagtgctgcttgctgctgg

SEQ ID NO: 89 - DNA, 23 bp, Homo sapiens
gcccctgcgtgggcccaagctgg

SEQ ID NO: 90 - DNA, 23 bp, Homo sapiens
gagtggccagagtccagcttggg

SEQ ID NO: 91 - DNA, 23 bp, Homo sapiens
ggcctccccaaagcctggccagg

SEQ ID NO: 92 - DNA, 23 bp, Homo sapiens
ggggccgagattgggtgttcagg

SEQ ID NO: 93 - DNA, 23 bp, Homo sapiens
gtggcgagaggggccgagattgg

SEQ ID NO: 94 - DNA, 23 bp, Homo sapiens
gagtgccgccgaggcggggcggg

SEQ ID NO: 95 - DNA, 23 bp, Homo sapiens
ggagtgccgccgaggcggggcgg

SEQ ID NO: 96 - DNA, 23 bp, Homo sapiens
ggagaggagtgccgccgaggcgg

SEQ ID NO: 97 - DNA, 21 bp, Artificial Sequence
  source: /note="Description of Artificial Sequence: Synthetic primer"
aaaaccacccttctctctggc

SEQ ID NO: 98 - DNA, 21 bp, Artificial Sequence
  source: /note="Description of Artificial Sequence: Synthetic primer"
ggagattggagacacggagag

SEQ ID NO: 99 - DNA, 20 bp, Artificial Sequence
  source: /note="Description of Artificial Sequence: Synthetic primer"
ccatccccttctgtgaatgt

SEQ ID NO: 100 - DNA, 20 bp, Artificial Sequence
  source: /note="Description of Artificial Sequence: Synthetic primer"
ggagattggagacacggaga

SEQ ID NO: 101 - DNA, 20 bp, Artificial Sequence
  source: /note="Description of Artificial Sequence: Synthetic primer"
ctggaaagccaatgcctgac

SEQ ID NO: 102 - DNA, 20 bp, Artificial Sequence
  source: /note="Description of Artificial Sequence: Synthetic primer"
ggcagcaaactccttgtcct

SEQ ID NO: 103 - DNA, 20 bp, Artificial Sequence
  source: /note="Description of Artificial Sequence: Synthetic primer"
aagcaccgactcggtgccac

SEQ ID NO: 104 - DNA, 20 bp, Artificial Sequence
  source: /note="Description of Artificial Sequence: Synthetic primer"
tcacctccaatgactagggg

SEQ ID NO: 105 - DNA, 22 bp, Artificial Sequence
  source: /note="Description of Artificial Sequence: Synthetic primer"
caagttgataacggactagcct

SEQ ID NO: 106 - DNA, 23 bp, Artificial Sequence
  source: /note="Description of Artificial Sequence: Synthetic primer"
agtccgagcagaagaagaagttt

SEQ ID NO: 107 - DNA, 25 bp, Artificial Sequence
  source: /note="Description of Artificial Sequence: Synthetic primer"
tttcaagttgataacggactagcct

SEQ ID NO: 108 - DNA, 20 bp, Artificial Sequence
  source: /note="Description of Artificial Sequence: Synthetic primer"
aaacagcagattcgcctgga

SEQ ID NO: 109 - DNA, 20 bp, Artificial Sequence
  source: /note="Description of Artificial Sequence: Synthetic primer"
tcatccgctcgatgaagctc

SEQ ID NO: 110 - DNA, 20 bp, Artificial Sequence
  source: /note="Description of Artificial Sequence: Synthetic primer"
tccaaaatcaagtggggcga

SEQ ID NO: 111 - DNA, 20 bp, Artificial Sequence
  source: /note="Description of Artificial Sequence: Synthetic primer"
tgatgacccttttggctccc

SEQ ID NO: 112 - DNA, 45 bp, Artificial Sequence
  source: /note="Description of Artificial Sequence: Synthetic primer"
gaggaattctttttttgttygaatatgttggaggttttttggaag

SEQ ID NO: 113 - DNA, 42 bp, Artificial Sequence
  source: /note="Description of Artificial Sequence: Synthetic primer"
gagaagcttaaataaaaaacracaatactcaacccaacaacc

SEQ ID NO: 114 - DNA, 17 bp, Artificial Sequence
  source: /note="Description of Artificial Sequence: Synthetic primer"
caggaaacagctatgac

SEQ ID NO: 115 - DNA, 39 bp, Artificial Sequence
  source: /note="Description of Artificial Sequence: Synthetic primer"
gcctctagaggtacctgagggcctatttcccatgattcc

SEQ ID NO: 116 - DNA, 133 bp, Artificial Sequence
  source: /note="Description of Artificial Sequence: Synthetic primer"
  modified_base (92)..(111): a, c, t, g, unknown or other
acctctagaaaaaaagcaccgactcggtgccactttttcaagttgataacggactagccttattttaacttgctatttctagctctaaaacnnnnnnnnnnnnnnnnnnnnggtgtttcgtcctttccacaag

SEQ ID NO: 117 - DNA, 133 bp, Artificial Sequence
  source: /note="Description of Artificial Sequence: Synthetic primer"
  modified_base (92)..(111): a, c, t, g, unknown or other
acctctagaaaaaaagcaccgactcggtgccactttttcaagttgataacggactagccttatattaacttgctatttctagctctaatacnnnnnnnnnnnnnnnnnnnnggtgtttcgtcctttccacaag

SEQ ID NO: 118 - DNA, 153 bp, Artificial Sequence
  source: /note="Description of Artificial Sequence: Synthetic primer"
  modified_base (112)..(131): a, c, t, g, unknown or other
acctctagaaaaaaagcaccgactcggtgccactttttcaagttgataacggactagccttattttaacttgctatgctgttttgtttccaaaacagcatagctctaaaacnnnnnnnnnnnnnnnnnnnnggtgtttcgtcctttccacaag

SEQ ID NO: 119 - DNA, 153 bp, Artificial Sequence
  source: /note="Description of Artificial Sequence: Synthetic primer"
  modified_base (112)..(131): a, c, t, g, unknown or other
acctctagaaaaaaagcaccgactcggtgccactttttcaagttgataacggactagccttatattaacttgctatgctgtattgtttccaatacagcatagctctaatacnnnnnnnnnnnnnnnnnnnnggtgtttcgtcctttccacaag

SEQ ID NO: 120 - DNA, 335 bp, Artificial Sequence
  source: /note="Description of Artificial Sequence: Synthetic polynucleotide"
gagggcctatttcccatgattccttcatatttgcatatacgatacaaggctgttagagagataattggaattaatttgactgtaaacacaaagatattagtacaaaatacgtgacgtagaaagtaataatttcttgggtagtttgcagttttaaaattatgttttaaaatggactatcatatgcttaccgtaacttgaaagtatttcgatttcttggctttatatatcttgtggaaaggacgaaacaccggaaccattcaaaacagcatagcaagttaaaataaggctagtccgttatcaacttgaaaaagtggcaccgagtcggtgcttttttt

SEQ ID NO: 121 - DNA, 360 bp, Artificial Sequence
  source: /note="Description of Artificial Sequence: Synthetic polynucleotide"
  modified_base (288)..(317): a, c, t, g, unknown or other
gagggcctatttcccatgattccttcatatttgcatatacgatacaaggctgttagagagataattggaattaatttgactgtaaacacaaagatattagtacaaaatacgtgacgtagaaagtaataatttcttgggtagtttgcagttttaaaattatgttttaaaatggactatcatatgcttaccgtaacttgaaagtatttcgatttcttggctttatatatcttgtggaaaggacgaaacaccgggttttagagctatgctgttttgaatggtcccaaaacnnnnnnnnnnnnnnnnnnnnnnnnnnnnnngttttagagctatgctgttttgaatggtcccaaaacttttttt

SEQ ID NO: 122 - DNA, 318 bp, Artificial Sequence
  source: /note="Description of Artificial Sequence: Synthetic polynucleotide"
  modified_base (250)..(269): a, c, t, g, unknown or other
gagggcctatttcccatgattccttcatatttgcatatacgatacaaggctgttagagagataattggaattaatttgactgtaaacacaaagatattagtacaaaatacgtgacgtagaaagtaataatttcttgggtagtttgcagttttaaaattatgttttaaaatggactatcatatgcttaccgtaacttgaaagtatttcgatttcttggctttatatatcttgtggaaaggacgaaacaccnnnnnnnnnnnnnnnnnnnngttttagagctagaaatagcaagttaaaataaggctagtccgttttttt

SEQ ID NO: 123 - DNA, 325 bp, Artificial Sequence
  source: /note="Description of Artificial Sequence: Synthetic polynucleotide"
  modified_base (250)..(269): a, c, t, g, unknown or other
gagggcctatttcccatgattccttcatatttgcatatacgatacaaggctgttagagagataattggaattaatttgactgtaaacacaaagatattagtacaaaatacgtgacgtagaaagtaataatttcttgggtagtttgcagttttaaaattatgttttaaaatggactatcatatgcttaccgtaacttgaaagtatttcgatttcttggctttatatatcttgtggaaaggacgaaacaccnnnnnnnnnnnnnnnnnnnngttttagagctagaaatagcaagttaaaataaggctagtccgttatcatttttttt

SEQ ID NO: 124 - DNA, 337 bp, Artificial Sequence
  source: /note="Description of Artificial Sequence: Synthetic polynucleotide"
  modified_base (250)..(269): a, c, t, g, unknown or other
gagggcctatttcccatgattccttcatatttgcatatacgatacaaggctgttagagagataattggaattaatttgactgtaaacacaaagatattagtacaaaatacgtgacgtagaaagtaataatttcttgggtagtttgcagttttaaaattatgttttaaaatggactatcatatgcttaccgtaacttgaaagtatttcgatttcttggctttatatatcttgtggaaaggacgaaacaccnnnnnnnnnnnnnnnnnnnngttttagagctagaaatagcaagttaaaataaggctagtccgttatcaacttgaaaaagtgttttttt

SEQ ID NO: 125 - DNA, 352 bp, Artificial Sequence
  source: /note="Description of Artificial Sequence: Synthetic polynucleotide"
  modified_base (250)..(269): a, c, t, g, unknown or other
gagggcctatttcccatgattccttcatatttgcatatacgatacaaggctgttagagagataattggaattaatttgactgtaaacacaaagatattagtacaaaatacgtgacgtagaaagtaataatttcttgggtagtttgcagttttaaaattatgttttaaaatggactatcatatgcttaccgtaacttgaaagtatttcgatttcttggctttatatatcttgtggaaaggacgaaacaccnnnnnnnnnnnnnnnnnnnngttttagagctagaaatagcaagttaaaataaggctagtccgttatcaacttgaaaaagtggcaccgagtcggtgcttttttt

SEQ ID NO: 126 - DNA, 5101 bp, Artificial Sequence
  source: /note="Description of Artificial Sequence: Synthetic polynucleotide"
cgttacataacttacggtaaatggcccgcctggctgaccgcccaacgacccccgcccattgacgtcaataatgacgtatgttcccatagtaacgccaatagggactttccattgacgtcaatgggtggagtatttacggtaaactgcccacttggcagtacatcaagtgtatcatatgccaagtacgccccctattgacgtcaatgacggtaaatggcccgcctggcattatgcccagtacatgaccttatgggactttcctacttggcagtacatctacgtattagtcatcgctattaccatggtcgaggtgagccccacgttctgcttcactctccccatctcccccccctccccacccccaattttgtatttatttattttttaattattttgtgcagcgatgggggcggggggggggggggggcgcgcgccaggcggggcggggcggggcgaggggcggggcggggcgaggcggagaggtgcggcggcagccaatcagagcggcgcgctccgaaagtttccttttatggcgaggcggcggcggcggcggccctataaaaagcgaagcgcgcggcgggcgggagtcgctgcgacgctgccttcgccccgtgccccgctccgccgccgcctcgcgccgcccgccccggctctgactgaccgcgttactcccacaggtgagcgggcgggacggcccttctcctccgggctgtaattagctgagcaagaggtaagggtttaagggatggttggttggtggggtattaatgtttaattacctggagcacctgcctgaaatcactttttttcaggttggaccggtgccaccatggactataaggaccacgacggagactacaaggatcatgatattgattacaaagacgatgacgataagatggccccaaagaagaagcggaaggtcggtatccacggagtcccagcagccgacaagaagtacagcatcggcctggacatcggcaccaactctgtgggctgggccgtgatcaccgacgagtacaaggtgcccagcaagaaattcaaggtgctgggcaacaccgaccggcacagcatcaagaagaacctgatcggagccctgctgttcgacagcggcgaaacagccgaggccacccggctgaagagaaccgccagaagaagatacaccagacggaagaaccggatctgctatctgcaagagatcttcagcaacgagatggccaaggtggacgacagcttcttccacagactggaagagtccttcctggtggaagaggataagaagcacgagcggcaccccatcttcggcaacatcgtggacgaggtggcctaccacgagaagtaccccaccatctaccacctgagaaagaaactggtggacagcaccgacaaggccgacctgcggctgatctatctggccctggcccacatgatcaagttccggggccacttcctgatcgagggcgacctgaaccccgacaacagcgacgtggacaagctgttcatccagctggtgcagacctacaaccagctgttcgaggaaaaccccatcaacgccagcggcgtggacgccaaggccatcctgtctgccagactgagcaagagcagacggctggaaaatctgatcgcccagctgcccggcgagaagaagaatggcctgttcggcaacctgattgccctgagcctgggcctgacccccaacttcaagagcaacttcgacctggccgaggatgccaaactgcagctgagcaaggacacctacgacgacgacctggacaacctgctggcccagatcggcgaccagtacgccgacctgtttctggccgccaagaacctgtccgacgccatcctgctgagcgacatcctgagagtgaacaccgagatcaccaaggcccccctgagcgcctctatgatcaagagatacgacgagcaccaccaggacctgaccctgctgaaagctctcgtgcggcagcagctgcctgagaagtacaaagagattttcttcgaccagagcaagaacggctacgccggctacattgacggcggagccagccaggaagagttctacaagttcatcaagcccatcctggaaaagatggacggcaccgaggaactgctcgtgaagctgaacagagaggacctgctgcggaagcagcggaccttcgacaacggcagcatcccccaccagatccacctgggagagctgcacgccattctgcggcggcaggaagatttttacccattcctgaaggacaaccgggaaaagatcgagaagatcctgaccttccgcatcccctactacgtgggccctctggccaggggaaacagcagattcgcctggatgaccagaaagagcgaggaaaccatcaccccctggaacttcgaggaagtggtggacaagggcgcttccgcccagagcttcatcgagcggatgaccaacttcgataagaacctgcccaacgagaaggtgctgcccaagcacagcctgctgtacgagtacttcaccgtgtataacgagctgaccaaagtgaaatacgtgaccgagggaatgagaaagcccgccttcctgagcggcgagcagaaaaaggccatcgtggacctgctgttcaagaccaaccggaaagtgaccgtgaagcagctgaaagaggactacttcaagaaaatcgagtgcttcgactccgtggaaatctccggcgtggaagatcggttcaacgcctccctgggcacataccacgatctgctgaaaattatcaaggacaaggacttcctggacaatgaggaaaacgaggacattctggaagatatcgtgctgaccctgacactgtttgaggacagagagatgatcgaggaacggctgaaaacctatgcccacctgttcgacgacaaagtgatgaagcagctgaagcggcggagatacaccggctggggcaggctgagccggaagctgatcaacggcatccgggacaagcagtccggcaagacaatcctggatttcctgaagtccgacggcttcgccaacagaaacttcatgcagctgatccacgacgacagcctgacctttaaagaggacatccagaaagcccaggtgtccggccagggcgatagcctgcacgagcacattgccaatctggccggcagccccgccattaagaagggcatcctgcagacagtgaaggtggtggacgagctcgtgaaagtgatgggccggcacaagcccgagaacatcgtgatcgaaatggccagagagaaccagaccacccagaagggacagaagaacagccgcgagagaatgaagcggatcgaagagggcatcaaagagctgggcagccagatcctgaaagaacaccccgtggaaaacacccagctgcagaacgagaagctgtacctgtactacctgcagaatgggcgggatatgtacgtggaccaggaactggacatcaaccggctgtccgactacgatgtggaccatatcgtgcctcagagctttctgaaggacgactccatcgacaacaaggtgctgaccagaagcgacaagaaccggggcaagagcgacaacgtgccctccgaagaggtcgtgaagaagatgaagaactactggcggcagctgctgaacgccaagctgattacccagagaaagttcgacaatctgaccaaggccgagagaggcggcctgagcgaactggataaggccggcttcatcaagagacagctggtggaaacccggcagatcacaaagcacgtggcacagatcctggactcccggatgaacactaagtacgacgagaatgacaagctgatccgggaagtgaaagtgatcaccctgaagtccaagctggtgtccgatttccggaaggatttccagttttacaaagtgcgcgagatcaacaactaccaccacgcccacgacgcctacctgaacgccgtcgtgggaaccgccctgatcaaaaagtaccctaagctggaaagcgagttcgtgtacggcgactacaaggtgtacgacgtgcggaagatgatcgccaagagcgagcaggaaatcggcaaggctaccgccaagtacttcttctacagcaacatcatgaactttttcaagaccgagattaccctggccaacggcgagatccggaagcggcctctgatcgagacaaacggcgaaaccggggagatcgtgtgggataagggccgggattttgccaccgtgcggaaagtgctgagcatgccccaagtgaatatcgtgaaaaagaccgaggtgcagacaggcggcttcagcaaagagtctatcctgcccaagaggaacagcgataagctgatcgccagaaagaaggactgggaccctaagaagtacggcggcttcgacagccccaccgtggcctattctgtgctggtggtggccaaagtggaaaagggcaagtccaagaaactgaagagtgtgaaagagctgctggggatcaccatcatggaaagaagcagcttcgagaagaatcccatcgactttctggaagccaagggctacaaagaagtgaaaaaggacctgatcatcaagctgcctaagtactccctgttcgagctggaaaacggccggaagagaatgctggcctctgccggcgaactgcagaagggaaacgaactggccctgccctccaaatatgtgaacttcctgtacctggccagccactatgagaagctgaagggctcccccgaggataatgagcagaaacagctgtttgtggaacagcacaagcactacctggacgagatcatcgagcagatcagcgagttctccaagagagtgatcctggccgacgctaatctggacaaagtgctgtccgcctacaacaagcaccgggataagcccatcagagagcaggccgagaatatcatccacctgtttaccctgaccaatctgggagcccctgccgccttcaagtactttgacaccaccatcgaccggaagaggtacaccagcaccaaagaggtgctggacgccaccctgatccaccagagcatcaccggcctgtacgagacacggatcgacctgtctcagctgggaggcgactttctttttcttagcttgaccagctttcttagtagcagcaggacgctttaa

SEQ ID NO: 127 - DNA, 123 bp, Artificial Sequence
  source: /note="Description of Artificial Sequence: Synthetic polynucleotide"
ccaatggggaggacatcgatgtcacctccaatgactagggtgggcaaccacaaacccacgagggcagagtgctgcttgctgctggccaggcccctgcgtgggcccaagctggactctggccac

SEQ ID NO: 128 - DNA, 121 bp, Artificial Sequence
  source: /note="Description of Artificial Sequence: Synthetic polynucleotide"
cgagcagaagaagaagggctcccatcacatcaaccggtggcgcattgccacgaagcaggccaatggggaggacatcgatgtcacctccaatgactagggtgggcaaccacaaacccacgag

SEQ ID NO: 129 - DNA, 128 bp, Artificial Sequence
  source: /note="Description of Artificial Sequence: Synthetic polynucleotide"
ggaggacaaagtacaaacggcagaagctggaggaggaagggcctgagtccgagcagaagaagaagggctcccatcacatcaaccggtggcgcattgccacgaagcaggccaatggggaggacatcgat

SEQ ID NO: 130 - DNA, 130 bp, Artificial Sequence
  source: /note="Description of Artificial Sequence: Synthetic polynucleotide"
agaagctggaggaggaagggcctgagtccgagcagaagaagaagggctcccatcacatcaaccggtggcgcattgccacgaagcaggccaatggggaggacatcgatgtcacctccaatgactagggtgg

SEQ ID NO: 131 - DNA, 125 bp, Artificial Sequence
  source: /note="Description of Artificial Sequence: Synthetic polynucleotide"
cctcagtcttcccatcaggctctcagctcagcctgagtgttgaggccccagtggctgctctgggggcctcctgagtttctcatctgtgcccctccctccctggcccaggtgaaggtgtggttcca

SEQ ID NO: 132 - DNA, 129 bp, Artificial Sequence
  source: /note="Description of Artificial Sequence: Synthetic polynucleotide"
tcatctgtgcccctccctccctggcccaggtgaaggtgtggttccagaaccggaggacaaagtacaaacggcagaagctggaggaggaagggcctgagtccgagcagaagaagaagggctcccatcaca

SEQ ID NO: 133 - DNA, 129 bp, Artificial Sequence
  source: /note="Description of Artificial Sequence: Synthetic polynucleotide"
ctccaatgactagggtgggcaaccacaaacccacgagggcagagtgctgcttgctgctggccaggcccctgcgtgggcccaagctggactctggccactccctggccaggctttggggaggcctggagt

SEQ ID NO: 134 - DNA, 127 bp, Artificial Sequence
  source: /note="Description of Artificial Sequence: Synthetic polynucleotide"
ctgcttgctgctggccaggcccctgcgtgggcccaagctggactctggccactccctggccaggctttggggaggcctggagtcatggccccacagggcttgaagcccggggccgccattgacagag

SEQ ID NO: 135 - DNA, 25 bp, Artificial Sequence
  source: /note="Description of Artificial Sequence: Synthetic primer"
gaaattaatacgactcactataggg

SEQ ID NO: 136 - DNA, 126 bp, Artificial Sequence
  source: /note="Description of Artificial Sequence: Synthetic polynucleotide"
aaaaaagcaccgactcggtgccactttttcaagttgataacggactagccttattttaacttgctatttctagctctaaaacaacgacgagcgtgacaccaccctatagtgagtcgtattaatttc

SEQ ID NO: 137 - DNA, 126 bp, Artificial Sequence
  source: /note="Description of Artificial Sequence: Synthetic polynucleotide"
aaaaaagcaccgactcggtgccactttttcaagttgataacggactagccttattttaacttgctatttctagctctaaaacgcaacaattaatagactggacctatagtgagtcgtattaatttc

SEQ ID NO: 138 - DNA, 102 bp, Artificial Sequence
  source: /note="Description of Artificial Sequence: Synthetic polynucleotide"
gttttagagctatgctgttttgaatggtcccaaaacggaagggcctgagtccgagcagaagaagaagttttagagctatgctgttttgaatggtcccaaaac

SEQ ID NO: 139 - DNA, 100 bp, Homo sapiens
cggaggacaaagtacaaacggcagaagctggaggaggaagggcctgagtccgagcagaagaagaagggctcccatcacatcaaccggtggcgcattgcca

SEQ ID NO: 140 - DNA, 50 bp, Homo sapiens
agctggaggaggaagggcctgagtccgagcagaagaagaagggctcccac

SEQ ID NO: 141 - RNA, 30 nt, Artificial Sequence
  source: /note="Description of Artificial Sequence: Synthetic oligonucleotide"
gaguccgagcagaagaagaaguuuuagagc

SEQ ID NO: 142 - DNA, 49 bp, Homo sapiens
agctggaggaggaagggcctgagtccgagcagaagagaagggctcccat

SEQ ID NO: 143 - DNA, 53 bp, Homo sapiens
ctggaggaggaagggcctgagtccgagcagaagaagaagggctcccatcacat

SEQ ID NO: 144 - DNA, 52 bp, Homo sapiens
ctggaggaggaagggcctgagtccgagcagaagagaagggctcccatcacat

SEQ ID NO: 145 - DNA, 54 bp, Homo sapiens
ctggaggaggaagggcctgagtccgagcagaagaaagaagggctcccatcacat

SEQ ID NO: 146 - DNA, 50 bp, Homo sapiens
ctggaggaggaagggcctgagtccgagcagaagaagggctcccatcacat

SEQ ID NO: 147 - DNA, 47 bp, Homo sapiens
ctggaggaggaagggcctgagcccgagcagaagggctcccatcacat

SEQ ID NO: 148 - DNA, 23 bp, Homo sapiens
gtcacctccaatgactagggtgg

SEQ ID NO: 149 - DNA, 23 bp, Homo sapiens
gcgccaccggttgatgtgatggg

SEQ ID NO: 150 - RNA, 99 nt, Artificial Sequence
  source: /note="Description of Artificial Sequence: Synthetic oligonucleotide"
  modified_base (1)..(20): a, c, u, g, unknown or other
nnnnnnnnnnnnnnnnnnnnguuuuagagcuagaaauagcaaguuaaaauaaggcuaguccguuaucaacuugaaaaaguggcaccgagucggugcuuu

SEQ ID NO: 151 - DNA, 64 bp, Homo sapiens
caagaggcttgagtaggagaggagtgccgccgaggcggggcggggcggggcgtggagctgggct

SEQ ID NO: 152 - RNA, 20 nt, Artificial Sequence
  source: /note="Description of Artificial Sequence: Synthetic oligonucleotide"
gucaccuccaaugacuaggg

SEQ ID NO: 153 - RNA, 20 nt, Artificial Sequence
  source: /note="Description of Artificial Sequence: Synthetic oligonucleotide"
gucaccuccaaugacuaaga

SEQ ID NO: 154 - RNA, 20 nt, Artificial Sequence
  source: /note="Description of Artificial Sequence: Synthetic oligonucleotide"
gucaccuccaaugauuagga

SEQ ID NO: 155 - RNA, 20 nt, Artificial Sequence
  source: /note="Description of Artificial Sequence: Synthetic oligonucleotide"
gucaccuccagugacuagga

SEQ ID NO: 156 - RNA, 20 nt, Artificial Sequence
  source: /note="Description of Artificial Sequence: Synthetic oligonucleotide"
gucacuuccaaugacuagga

SEQ ID NO: 157 - RNA, 20 nt, Artificial Sequence
  source: /note="Description of Artificial Sequence: Synthetic oligonucleotide"
aucaccuccaaugacuagga

SEQ ID NO: 158 - RNA, 20 nt, Artificial Sequence
  source: /note="Description of Artificial Sequence: Synthetic oligonucleotide"
gucaccuccaaugaccaagg

SEQ ID NO: 159 - RNA, 20 nt, Artificial Sequence
  source: /note="Description of Artificial Sequence: Synthetic oligonucleotide"
gucaccuccaauaacuaagg

SEQ ID NO: 160 - RNA, 20 nt, Artificial Sequence
  source: /note="Description of Artificial Sequence: Synthetic oligonucleotide"
gucaccucuaaugacuaagg

SEQ ID NO: 161 - RNA, 20 nt, Artificial Sequence
  source: /note="Description of Artificial Sequence: Synthetic oligonucleotide"
gucgccuccaaugacuaagg

SEQ ID NO: 162 - RNA, 20 nt, Artificial Sequence
  source: /note="Description of Artificial Sequence: Synthetic oligonucleotide"
gucaccuccaauggccaggg

SEQ ID NO: 163 - RNA, 20 nt, Artificial Sequence
  source: /note="Description of Artificial Sequence: Synthetic oligonucleotide"
gucaccuccagugaccaggg

SEQ ID NO: 164 - RNA, 20 nt, Artificial Sequence
  source: /note="Description of Artificial Sequence: Synthetic oligonucleotide"
gucacccccaaugaccaggg

SEQ ID NO: 165 - RNA, 20 nt, Artificial Sequence
  source: /note="Description of Artificial Sequence: Synthetic oligonucleotide"
gccaccuccaaugaccaggg

SEQ ID NO: 166 - RNA, 20 nt, Artificial Sequence
  source: /note="Description of Artificial Sequence: Synthetic oligonucleotide"
gucaccuccaaugaccaaga

SEQ ID NO: 167 - RNA, 20 nt, Artificial Sequence
  source: /note="Description of Artificial Sequence: Synthetic oligonucleotide"
gucaccuccaauggcuggga

SEQ ID NO: 168 - RNA, 20 nt, Artificial Sequence
  source: /note="Description of Artificial Sequence: Synthetic oligonucleotide"
gucaccuccaacgaccagga

SEQ ID NO: 169 - RNA, 20 nt, Artificial Sequence
  source: /note="Description of Artificial Sequence: Synthetic oligonucleotide"
gucaccuccgaugauuagga

SEQ ID NO: 170 - RNA, 20 nt, Artificial Sequence
  source: /note="Description of Artificial Sequence: Synthetic oligonucleotide"
gucaccuccaauggccaagg

SEQ ID NO: 171 - RNA, 20 nt, Artificial Sequence
  source: /note="Description of Artificial Sequence: Synthetic oligonucleotide"
gucaccuccaacgauuaagg

SEQ ID NO: 172 - RNA, 20 nt, Artificial Sequence
  source: /note="Description of Artificial Sequence: Synthetic oligonucleotide"
gucaccuccgauggcuaagg

SEQ ID NO: 173 - RNA, 20 nt, Artificial Sequence
  source: /note="Description of Artificial Sequence: Synthetic oligonucleotide"
gucaccuucaauaacuaagg

SEQ ID NO: 174 - RNA, 20 nt, Artificial Sequence
  source: /note="Description of Artificial Sequence: Synthetic oligonucleotide"
gucaccuccaauggccaaga

SEQ ID NO: 175 - RNA, 20 nt, Artificial Sequence
  source: /note="Description of Artificial Sequence: Synthetic oligonucleotide"
gucaccuccaguggcuggga

SEQ ID NO: 176 - RNA, 20 nt, Artificial Sequence
  source: /note="Description of Artificial Sequence: Synthetic oligonucleotide"
gucaccuucaacgaccagga

SEQ ID NO: 177 - RNA, 20 nt, Artificial Sequence
  source: /note="Description of Artificial Sequence: Synthetic oligonucleotide"
gucaucuccgaugauuagga

SEQ ID NO: 178 - RNA, 20 nt, Artificial Sequence
  source: /note="Description of Artificial Sequence: Synthetic oligonucleotide"
gccaccuucaauggcuagga

SEQ ID NO: 179 - RNA, 20 nt, Artificial Sequence
  source: /note="Description of Artificial Sequence: Synthetic oligonucleotide"
gucaccuccaaugacuagaa

SEQ ID NO: 180 - RNA, 20 nt, Artificial Sequence
  source: /note="Description of Artificial Sequence: Synthetic oligonucleotide"
gucaccuccaaugacugagg

SEQ ID NO: 181 - RNA, 20 nt, Artificial Sequence
  source: /note="Description of Artificial Sequence: Synthetic oligonucleotide"
gucaccuccaaugaucaggg

SEQ ID NO: 182 - RNA, 20 nt, Artificial Sequence
  source: /note="Description of Artificial Sequence: Synthetic oligonucleotide"
gucaccuccaauagcuaggg

SEQ ID NO: 183 - RNA, 20 nt, Artificial Sequence
  source: /note="Description of Artificial Sequence: Synthetic oligonucleotide"
gucaccuccagcgacuaggg

SEQ ID NO: 184 - RNA, 20 nt, Artificial Sequence
  source: /note="Description of Artificial Sequence: Synthetic oligonucleotide"
gucaccucugaugacuaggg

SEQ ID NO: 185 - RNA, 20 nt, Artificial Sequence
  source: /note="Description of Artificial Sequence: Synthetic oligonucleotide"
gucacccucaaugacuaggg

SEQ ID NO: 186 - RNA, 20 nt, Artificial Sequence
  source: /note="Description of Artificial Sequence: Synthetic oligonucleotide"
gucauuuccaaugacuaggg

SEQ ID NO: 187 - RNA, 20 nt, Artificial Sequence
  source: /note="Description of Artificial Sequence: Synthetic oligonucleotide"
guugccuccaaugacuaggg

SEQ ID NO: 188 - RNA, 20 nt, Artificial Sequence
  source: /note="Description of Artificial Sequence: Synthetic oligonucleotide"
accaccuccaaugacuaggg

SEQ ID NO: 189 - RNA, 20 nt, Artificial Sequence
  source: /note="Description of Artificial Sequence: Synthetic oligonucleotide"
gucaccuccaaugacugaag

SEQ ID NO: 190 - RNA, 20 nt, Artificial Sequence
  source: /note="Description of Artificial Sequence: Synthetic oligonucleotide"
gucaccuccaauggucaggg

SEQ ID NO: 191 - RNA, 20 nt, Artificial Sequence
  source: /note="Description of Artificial Sequence: Synthetic oligonucleotide"
gucaccuccagcaacuaggg

SEQ ID NO: 192 - RNA, 20 nt, Artificial Sequence
  source: /note="Description of Artificial Sequence: Synthetic oligonucleotide"
gucaccuuugaugacuaggg

SEQ ID NO: 193 - RNA, 20 nt, Artificial Sequence
  source: /note="Description of Artificial Sequence: Synthetic oligonucleotide"
gucauucccaaugacuaggg

SEQ ID NO: 194 - RNA, 20 nt, Artificial Sequence
  source: /note="Description of Artificial Sequence: Synthetic oligonucleotide"
gcugccuccaaugacuaggg

SEQ ID NO: 195 - RNA, 20 nt, Artificial Sequence
  source: /note="Description of Artificial Sequence: Synthetic oligonucleotide"
gucaccuccaaugaccgaaa

SEQ ID NO: 196 - RNA, 20 nt, Artificial Sequence
  source: /note="Description of Artificial Sequence: Synthetic oligonucleotide"
gucaccuccaauagucgggg

SEQ ID NO: 197 - RNA, 20 nt, Artificial Sequence
  source: /note="Description of Artificial Sequence: Synthetic oligonucleotide"
gucaccuccggcagcuaggg

SEQ ID NO: 198 - RNA, 20 nt, Artificial Sequence
  source: /note="Description of Artificial Sequence: Synthetic oligonucleotide"
gucacccuuggugacuaggg

SEQ ID NO: 199 - RNA, 20 nt, Artificial Sequence
  source: /note="Description of Artificial Sequence: Synthetic oligonucleotide"
gucguucucaaugacuaggg

SEQ ID NO: 200 - RNA, 20 nt, Artificial Sequence
  source: /note="Description of Artificial Sequence: Synthetic oligonucleotide"
acugucuccaaugacuaggg

SEQ ID NO: 201 - RNA, 20 nt, Artificial Sequence
  source: /note="Description of Artificial Sequence: Synthetic oligonucleotide"
gcgccaccgguugaugugau

SEQ ID NO: 202 - RNA, 20 nt, Artificial Sequence
  source: /note="Description of Artificial Sequence: Synthetic oligonucleotide"
gcgccaccgguugauguaac

SEQ ID NO: 203 - RNA, 20 nt, Artificial Sequence
  source: /note="Description of Artificial Sequence: Synthetic oligonucleotide"
gcgccaccgguugacgugac

SEQ ID NO: 204 - RNA, 20 nt, Artificial Sequence
  source: /note="Description of Artificial Sequence: Synthetic oligonucleotide"
gcgccaccggcugaugugac

SEQ ID NO: 205 - RNA, 20 nt, Artificial Sequence
  source: /note="Description of Artificial Sequence: Synthetic oligonucleotide"
gcgccgccgguugaugugac

SEQ ID NO: 206 - RNA, 20 nt, Artificial Sequence
  source: /note="Description of Artificial Sequence: Synthetic oligonucleotide"
acgccaccgguugaugugac

SEQ ID NO: 207 - RNA, 20 nt, Artificial Sequence
  source: /note="Description of Artificial Sequence: Synthetic oligonucleotide"
gcgccaccgguugauauaau

SEQ ID NO: 208 - RNA, 20 nt, Artificial Sequence
  source: /note="Description of Artificial Sequence: Synthetic oligonucleotide"
gcgccaccgguuaauguaau

SEQ ID NO: 209 - RNA, 20 nt, Artificial Sequence
  source: /note="Description of Artificial Sequence: Synthetic oligonucleotide"
gcgccaccaguugauguaau

SEQ ID NO: 210 - RNA, 20 nt, Artificial Sequence
  source: /note="Description of Artificial Sequence: Synthetic oligonucleotide"
gcgucaccgguugauguaau

SEQ ID NO: 211 - RNA, 20 nt, Artificial Sequence
  source: /note="Description of Artificial Sequence: Synthetic oligonucleotide"
gcgccaccgguugguaugau

SEQ ID NO: 212 - RNA, 20 nt, Artificial Sequence
  source: /note="Description of Artificial Sequence: Synthetic oligonucleotide"
gcgccaccggcugauaugau

SEQ ID NO: 213 - RNA, 20 nt, Artificial Sequence
  source: /note="Description of Artificial Sequence: Synthetic oligonucleotide"
gcgccaucgguugauaugau

SEQ ID NO: 214 - RNA, 20 nt, Artificial Sequence
  source: /note="Description of Artificial Sequence: Synthetic oligonucleotide"
gugccaccgguugauaugau

SEQ ID NO: 215 - RNA, 20 nt, Artificial Sequence
  source: /note="Description of Artificial Sequence: Synthetic oligonucleotide"
gcgccaccgguugauauaac

SEQ ID NO: 216 - RNA, 20 nt, Artificial Sequence
  source: /note="Description of Artificial Sequence: Synthetic oligonucleotide"
gcgccaccgguuggugcgac

SEQ ID NO: 217 - RNA, 20 nt, Artificial Sequence
  source: /note="Description of Artificial Sequence: Synthetic oligonucleotide"
gcgccaccggucgauaugac

SEQ ID NO: 218 - RNA, 20 nt, Artificial Sequence
  source: /note="Description of Artificial Sequence: Synthetic oligonucleotide"
gcgccaccgauugacgugac

SEQ ID NO: 219 - RNA, 20 nt, Artificial Sequence
  source: /note="Description of Artificial Sequence: Synthetic oligonucleotide"
gcgccaccgguugguauaau

SEQ ID NO: 220 - RNA, 20 nt, Artificial Sequence
  source: /note="Description of Artificial Sequence: Synthetic oligonucleotide"
gcgccaccggucgacguaau

SEQ ID NO: 221 - RNA, 20 nt, Artificial Sequence
  source: /note="Description of Artificial Sequence: Synthetic oligonucleotide"
gcgccaccgauugguguaau

SEQ ID NO: 222 - RNA, 20 nt, Artificial Sequence
  source: /note="Description of Artificial Sequence: Synthetic oligonucleotide"
gcgccacugguuaauguaau

SEQ ID NO: 223 - RNA, 20 nt, Artificial Sequence
  source: /note="Description of Artificial Sequence: Synthetic oligonucleotide"
gcgccaccgguugguauaac

SEQ ID NO: 224 - RNA, 20 nt, Artificial Sequence
  source: /note="Description of Artificial Sequence: Synthetic oligonucleotide"
gcgccaccggcuggugcgac

SEQ ID NO: 225 - RNA, 20 nt, Artificial Sequence
  source: /note="Description of Artificial Sequence: Synthetic oligonucleotide"
gcgccacuggucgauaugac

SEQ ID NO: 226 - RNA, 20 nt, Artificial Sequence
  source: /note="Description of Artificial Sequence: Synthetic oligonucleotide"
gcgcuaccgauugacgugac

SEQ ID NO: 227 - RNA, 20 nt, Artificial Sequence
  source: /note="Description of Artificial Sequence: Synthetic oligonucleotide"
gugccacugguuggugugac

SEQ ID NO: 228 - RNA, 20 nt, Artificial Sequence
  source: /note="Description of Artificial Sequence: Synthetic oligonucleotide"
gcgccaccgguugauguggc

SEQ ID NO: 229 - RNA, 20 nt, Artificial Sequence
  source: /note="Description of Artificial Sequence: Synthetic oligonucleotide"
gcgccaccgguugaugcaau

SEQ ID NO: 230 - RNA, 20 nt, Artificial Sequence
  source: /note="Description of Artificial Sequence: Synthetic oligonucleotide"
gcgccaccgguugacaugau

SEQ ID NO: 231 - RNA, 20 nt, Artificial Sequence
  source: /note="Description of Artificial Sequence: Synthetic oligonucleotide"
gcgccaccgguuagugugau

SEQ ID NO: 232 - RNA, 20 nt, Artificial Sequence
  source: /note="Description of Artificial Sequence: Synthetic oligonucleotide"
gcgccaccggccgaugugau

SEQ ID NO: 233 - RNA, 20 nt, Artificial Sequence
  source: /note="Description of Artificial Sequence: Synthetic oligonucleotide"
gcgccaccaauugaugugau

SEQ ID NO: 234 - RNA, 20 nt, Artificial Sequence
  source: /note="Description of Artificial Sequence: Synthetic oligonucleotide"
gcgccauugguugaugugau

SEQ ID NO: 235 - RNA, 20 nt, Artificial Sequence
  source: /note="Description of Artificial Sequence: Synthetic oligonucleotide"
gcgcugccgguugaugugau

SEQ ID NO: 236 - RNA, 20 nt, Artificial Sequence
  source: /note="Description of Artificial Sequence: Synthetic oligonucleotide"
gcaucaccgguugaugugau

SEQ ID NO: 237 - RNA, 20 nt, Artificial Sequence
  source: /note="Description of Artificial Sequence: Synthetic oligonucleotide"
augccaccgguugaugugau

SEQ ID NO: 238 - RNA, 20 nt, Artificial Sequence
  source: /note="Description of Artificial Sequence: Synthetic oligonucleotide"
gcgccaccgguugaugcagu

SEQ ID NO: 239 - RNA, 20 nt, Artificial Sequence
  source: /note="Description of Artificial Sequence: Synthetic oligonucleotide"
gcgccaccgguuggcaugau

SEQ ID NO: 240 - RNA, 20 nt, Artificial Sequence
  source: /note="Description of Artificial Sequence: Synthetic oligonucleotide"
gcgccaccggccaaugugau

SEQ ID NO: 241 - RNA, 20 nt, Artificial Sequence
  source: /note="Description of Artificial Sequence: Synthetic oligonucleotide"
gcgccacuaauugaugugau

SEQ ID NO: 242 - RNA, 20 nt, Artificial Sequence
  source: /note="Description of Artificial Sequence: Synthetic oligonucleotide"
gcgcugucgguugaugugau

SEQ ID NO: 243 - RNA, 20 nt, Artificial Sequence
  source: /note="Description of Artificial Sequence: Synthetic oligonucleotide"
guaucaccgguugaugugau

SEQ ID NO: 244 - RNA, 20 nt, Artificial Sequence
  source: /note="Description of Artificial Sequence: Synthetic oligonucleotide"
gcgccaccgguugauacagc

SEQ ID NO: 245 - RNA, 20 nt, Artificial Sequence
  source: /note="Description of Artificial Sequence: Synthetic oligonucleotide"
gcgccaccgguuagcacgau

SEQ ID NO: 246 - RNA, 20 nt, Artificial Sequence
  source: /note="Description of Artificial Sequence: Synthetic oligonucleotide"
gcgccaccgaccagugugau

SEQ ID NO: 247 - RNA, 20 nt, Artificial Sequence
  source: /note="Description of Artificial Sequence: Synthetic oligonucleotide"
gcgccauuaacugaugugau

SEQ ID NO: 248 - RNA, 20 nt, Artificial Sequence
  source: /note="Description of Artificial Sequence: Synthetic oligonucleotide"
gcguuguugguugaugugau

SEQ ID NO: 249 - RNA, 20 nt, Artificial Sequence
  source: /note="Description of Artificial Sequence: Synthetic oligonucleotide"
auauuaccgguugaugugau

SEQ ID NO: 250 - RNA, 20 nt, Artificial Sequence
  source: /note="Description of Artificial Sequence: Synthetic oligonucleotide"
gucaccuccaaugacuaggg

SEQ ID NO: 251 - RNA, 20 nt, Artificial Sequence
  source: /note="Description of Artificial Sequence: Synthetic oligonucleotide"
gucaccuggaaugacuaggg

SEQ ID NO: 252 - RNA, 20 nt, Artificial Sequence
  source: /note="Description of Artificial Sequence: Synthetic oligonucleotide"
gucacgaccaaugacuaggg

SEQ ID NO: 253 - RNA, 20 nt, Artificial Sequence
  source: /note="Description of Artificial Sequence: Synthetic oligonucleotide"
gucugcuccaaugacuaggg

SEQ ID NO: 254 - RNA, 20 nt, Artificial Sequence
  source: /note="Description of Artificial Sequence: Synthetic oligonucleotide"
gagaccuccaaugacuaggg

SEQ ID NO: 255 - RNA, 20 nt, Artificial Sequence
  source: /note="Description of Artificial Sequence: Synthetic oligonucleotide"
gucaccaggaaugacuaggg

SEQ ID NO: 256 - RNA, 20 nt, Artificial Sequence
  source: /note="Description of Artificial Sequence: Synthetic oligonucleotide"
gucugguccaaugacuaggg

SEQ ID NO: 257 - RNA, 20 nt, Artificial Sequence
  source: /note="Description of Artificial Sequence: Synthetic oligonucleotide"
gaguccuccaaugacuaggg

SEQ ID NO: 258 - RNA, 20 nt, Artificial Sequence
  source: /note="Description of Artificial Sequence: Synthetic oligonucleotide"
gucacgaggaaugacuaggg

SEQ ID NO: 259 - RNA, 20 nt, Artificial Sequence
  source: /note="Description of Artificial Sequence: Synthetic oligonucleotide"
gucuggaccaaugacuaggg

SEQ ID NO: 260 - RNA, 20 nt, Artificial Sequence
  source: /note="Description of Artificial Sequence: Synthetic oligonucleotide"
gagugcuccaaugacuaggg

SEQ ID NO: 261 - RNA, 20 nt, Artificial Sequence
  source: /note="Description of Artificial Sequence: Synthetic oligonucleotide"
gucugcuggaaugacuaggg

SEQ ID NO: 262 - RNA, 20 nt, Artificial Sequence
  source: /note="Description of Artificial Sequence: Synthetic oligonucleotide"
gagacgaccaaugacuaggg

SEQ ID NO: 263 - RNA, 20 nt, Artificial Sequence
  source: /note="Description of Artificial Sequence: Synthetic oligonucleotide"
gagaccuggaaugacuaggg

SEQ ID NO: 264 - DNA, 40 bp, Homo sapiens
ggacatcgatgtcacctccaatgactagggtgggcaacca

SEQ ID NO: 265 - RNA, 20 nt, Artificial Sequence
  source: /note="Description of Artificial Sequence: Synthetic oligonucleotide"
gucaccuccaaugacuaggg

SEQ ID NO: 266 - RNA, 20 nt, Artificial Sequence
  source: /note="Description of Artificial Sequence: Synthetic oligonucleotide"
  modified_base (20)..(20): a, c, u, g, unknown or other
gucaccuccaaugacuaggn

SEQ ID NO: 267 - RNA, 20 nt, Artificial Sequence
  source: /note="Description of Artificial Sequence: Synthetic oligonucleotide"
  modified_base (19)..(19): a, c, u, g, unknown or other
gucaccuccaaugacuagng

SEQ ID NO: 268 - RNA, 20 nt, Artificial Sequence
  source: /note="Description of Artificial Sequence: Synthetic oligonucleotide"
  modified_base (18)..(18): a, c, u, g, unknown or other
gucaccuccaaugacuangg

SEQ ID NO: 269 - RNA, 20 nt, Artificial Sequence
  source: /note="Description of Artificial Sequence: Synthetic oligonucleotide"
  modified_base (17)..(17): a, c, u, g, unknown or other
gucaccuccaaugacunggg

SEQ ID NO: 270 - RNA, 20 nt, Artificial Sequence
  source: /note="Description of Artificial Sequence: Synthetic oligonucleotide"
  modified_base (16)..(16): a, c, u, g, unknown or other
gucaccuccaaugacnaggg

SEQ ID NO: 271 - RNA, 20 nt, Artificial Sequence
  source: /note="Description of Artificial Sequence: Synthetic oligonucleotide"
  modified_base (15)..(15): a, c, u, g, unknown or other
gucaccuccaauganuaggg

SEQ ID NO: 272 - RNA, 20 nt, Artificial Sequence
  source: /note="Description of Artificial Sequence: Synthetic oligonucleotide"
  modified_base (14)..(14): a, c, u, g, unknown or other
gucaccuccaaugncuaggg

SEQ ID NO: 273 - RNA, 20 nt, Artificial Sequence
  source: /note="Description of Artificial Sequence: Synthetic oligonucleotide"
  modified_base (13)..(13): a, c, u, g, unknown or other
gucaccuccaaunacuaggg

SEQ ID NO: 274 - RNA, 20 nt, Artificial Sequence
  source: /note="Description of Artificial Sequence: Synthetic oligonucleotide"
  modified_base (12)..(12): a, c, u, g, unknown or other
gucaccuccaangacuaggg

SEQ ID NO: 275 - RNA, 20 nt, Artificial Sequence
  source: /note="Description of Artificial Sequence: Synthetic oligonucleotide"
  modified_base (11)..(11): a, c, u, g, unknown or other
gucaccuccanugacuaggg

SEQ ID NO: 276 - RNA, 20 nt, Artificial Sequence
  source: /note="Description of Artificial Sequence: Synthetic oligonucleotide"
  modified_base (10)..(10): a, c, u, g, unknown or other
gucaccuccnaugacuaggg

SEQ ID NO: 277 - RNA, 20 nt, Artificial Sequence
  source: /note="Description of Artificial Sequence: Synthetic oligonucleotide"
  modified_base (9)..(9): a, c, u, g, unknown or other
gucaccucnaaugacuaggg

SEQ ID NO: 278 - RNA, 20 nt, Artificial Sequence
  source: /note="Description of Artificial Sequence: Synthetic oligonucleotide"
  modified_base (8)..(8): a, c, u, g, unknown or other
gucaccuncaaugacuaggg

SEQ ID NO: 279 - RNA, 20 nt, Artificial Sequence
  source: /note="Description of Artificial Sequence: Synthetic oligonucleotide"
  modified_base (7)..(7): a, c, u, g, unknown or other
gucaccnccaaugacuaggg

SEQ ID NO: 280 - RNA, 20 nt, Artificial Sequence
  source: /note="Description of Artificial Sequence: Synthetic oligonucleotide"
  modified_base (6)..(6): a, c, u, g, unknown or other
gucacnuccaaugacuaggg

SEQ ID NO: 281 - RNA, 20 nt, Artificial Sequence
  source: /note="Description of Artificial Sequence: Synthetic oligonucleotide"
  modified_base (5)..(5): a, c, u, g, unknown or other
gucancuccaaugacuaggg

SEQ ID NO: 282 - RNA, 20 nt, Artificial Sequence
  source: /note="Description of Artificial Sequence: Synthetic oligonucleotide"
  modified_base (4)..(4): a, c, u, g, unknown or other
gucnccuccaaugacuaggg

SEQ ID NO: 283 - RNA, 20 nt, Artificial Sequence
  source: /note="Description of Artificial Sequence: Synthetic oligonucleotide"
  modified_base (3)..(3): a, c, u, g, unknown or other
gunaccuccaaugacuaggg

SEQ ID NO: 284 - RNA, 20 nt, Artificial Sequence
  source: /note="Description of Artificial Sequence: Synthetic oligonucleotide"
  modified_base (2)..(2): a, c, u, g, unknown or other
gncaccuccaaugacuaggg

SEQ ID NO: 285 - RNA, 20 nt, Artificial Sequence
  source: /note="Description of Artificial Sequence: Synthetic oligonucleotide"
gucaccuccaaugacuaggg

SEQ ID NO: 286 - RNA, 20 nt, Artificial Sequence
  source: /note="Description of Artificial Sequence: Synthetic oligonucleotide"
gacaucgauguccuccccau

SEQ ID NO: 287 - RNA, 20 nt, Artificial Sequence
  source: /note="Description of Artificial Sequence: Synthetic oligonucleotide"
gcgccaccgguugaugugau

SEQ ID NO: 288 - RNA, 20 nt, Artificial Sequence
  source: /note="Description of Artificial Sequence: Synthetic oligonucleotide"
gucaccuccaaugacuaggg

SEQ ID NO: 289 - RNA, 20 nt, Artificial Sequence
  source: /note="Description of Artificial Sequence: Synthetic oligonucleotide"
gucaccuccaaugacuagaa

SEQ ID NO: 290 - RNA, 20 nt, Artificial Sequence
  source: /note="Description of Artificial Sequence: Synthetic oligonucleotide"
gucaccuccaaugacugagg

SEQ ID NO: 291 - RNA, 20 nt, Artificial Sequence
  source: /note="Description of Artificial Sequence: Synthetic oligonucleotide"
gucaccuccaaugaucaggg

SEQ ID NO: 292 - RNA, 20 nt, Artificial Sequence
  source: /note="Description of Artificial Sequence: Synthetic oligonucleotide"
gucaccuccaauagcuaggg

SEQ ID NO: 293 - RNA, 20 nt, Artificial Sequence
  source: /note="Description of Artificial Sequence: Synthetic oligonucleotide"
gucaccuccagcgacuaggg

SEQ ID NO: 294 - RNA, 20 nt, Artificial Sequence
  source: /note="Description of Artificial Sequence: Synthetic oligonucleotide"
gucaccucugaugacuaggg

SEQ ID NO: 295 - RNA, 20 nt, Artificial Sequence
  source: /note="Description of Artificial Sequence: Synthetic oligonucleotide"
gucacccucaaugacuaggg

SEQ ID NO: 296 - RNA, 20 nt, Artificial Sequence
  source: /note="Description of Artificial Sequence: Synthetic oligonucleotide"
gucauuuccaaugacuaggg

SEQ ID NO: 297 - RNA, 20 nt, Artificial Sequence
  source: /note="Description of Artificial Sequence: Synthetic oligonucleotide"
guugccuccaaugacuaggg

SEQ ID NO: 298 - RNA, 20 nt, Artificial Sequence
  source: /note="Description of Artificial Sequence: Synthetic oligonucleotide"
accaccuccaaugacuaggg

SEQ ID NO: 299 - RNA, 20 nt, Artificial Sequence
  source: /note="Description of Artificial Sequence: Synthetic oligonucleotide"
gucaccuccaaugacugaag

SEQ ID NO: 300 - RNA, 20 nt, Artificial Sequence
  source: /note="Description of Artificial Sequence: Synthetic oligonucleotide"
gucaccuccaauggucaggg

SEQ ID NO: 301 - RNA, 20 nt, Artificial Sequence
  source: /note="Description of Artificial Sequence: Synthetic oligonucleotide"
gucaccuccagcaacuaggg

SEQ ID NO: 302 - RNA, 20 nt, Artificial Sequence
  source: /note="Description of Artificial Sequence: Synthetic oligonucleotide"
gucaccuuugaugacuaggg

SEQ ID NO: 303 - RNA, 20 nt, Artificial Sequence
  source: /note="Description of Artificial Sequence: Synthetic oligonucleotide"
gucauucccaaugacuaggg

SEQ ID NO: 304 - RNA, 20 nt, Artificial Sequence
  source: /note="Description of Artificial Sequence: Synthetic oligonucleotide"
gcugccuccaaugacuaggg

SEQ ID NO: 305 - RNA, 20 nt, Artificial Sequence
  source: /note="Description of Artificial Sequence: Synthetic oligonucleotide"
gucaccuccaaugaccgaaa

SEQ ID NO: 306 - RNA, 20 nt, Artificial Sequence
  source: /note="Description of Artificial Sequence: Synthetic oligonucleotide"
gucaccuccaauagucgggg

SEQ ID NO: 307 - RNA, 20 nt, Artificial Sequence
  source: /note="Description of Artificial Sequence: Synthetic oligonucleotide"
gucaccuccggcagcuaggg

SEQ ID NO: 308 - RNA, 20 nt, Artificial Sequence
  source: /note="Description of Artificial Sequence: Synthetic oligonucleotide"
gucacccuuggugacuaggg

SEQ ID NO: 309 - RNA, 20 nt, Artificial Sequence
  source: /note="Description of Artificial Sequence: Synthetic oligonucleotide"
gucguucucaaugacuaggg

SEQ ID NO: 310 - RNA, 20 nt, Artificial Sequence
  source: /note="Description of Artificial Sequence: Synthetic oligonucleotide"
acugucuccaaugacuaggg

SEQ ID NO: 311 - RNA, 20 nt, Artificial Sequence
  source: /note="Description of Artificial Sequence: Synthetic oligonucleotide"
gcgccaccgguugaugugau

SEQ ID NO: 312 - RNA, 20 nt, Artificial Sequence
  source: /note="Description of Artificial Sequence: Synthetic oligonucleotide"
gcgccaccgguugauguggc

SEQ ID NO: 313 - RNA, 20 nt, Artificial Sequence
  source: /note="Description of Artificial Sequence: Synthetic oligonucleotide"
gcgccaccgguugaugcaau

SEQ ID NO: 314 - RNA, 20 nt, Artificial Sequence
  source: /note="Description of Artificial Sequence: Synthetic oligonucleotide"
gcgccaccgguugacaugau

SEQ ID NO: 315 - RNA, 20 nt, Artificial Sequence
  source: /note="Description of Artificial Sequence: Synthetic oligonucleotide"
gcgccaccgguuagugugau

SEQ ID NO: 316 - RNA, 20 nt, Artificial Sequence
  source: /note="Description of Artificial Sequence: Synthetic oligonucleotide"
gcgccaccggccgaugugau

SEQ ID NO: 317 - RNA, 20 nt, Artificial Sequence
  source: /note="Description of Artificial Sequence: Synthetic oligonucleotide"
gcgccaccaauugaugugau

SEQ ID NO: 318 - RNA, 20 nt, Artificial Sequence
  source: /note="Description of Artificial Sequence: Synthetic oligonucleotide"
gcgccauugguugaugugau

SEQ ID NO: 319 - RNA, 20 nt, Artificial Sequence
  source: /note="Description of Artificial Sequence: Synthetic oligonucleotide"
gcgcugccgguugaugugau

SEQ ID NO: 320 - RNA, 20 nt, Artificial Sequence
  source: /note="Description of Artificial Sequence: Synthetic oligonucleotide"
gcaucaccgguugaugugau

SEQ ID NO: 321 - RNA, 20 nt, Artificial Sequence
  source: /note="Description of Artificial Sequence: Synthetic oligonucleotide"
augccaccgguugaugugau

SEQ ID NO: 322 - RNA, 20 nt, Artificial Sequence
  source: /note="Description of Artificial Sequence: Synthetic oligonucleotide"
gcgccaccgguugaugcagu

SEQ ID NO: 323 - RNA, 20 nt, Artificial Sequence
  source: /note="Description of Artificial Sequence: Synthetic oligonucleotide"
gcgccaccgguuggcaugau

SEQ ID NO: 324 - RNA, 20 nt, Artificial Sequence
  source: /note="Description of Artificial Sequence: Synthetic oligonucleotide"
gcgccaccggccaaugugau

SEQ ID NO: 325 - RNA, 20 nt, Artificial Sequence
  source: /note="Description of Artificial Sequence: Synthetic oligonucleotide"
gcgccacuaauugaugugau

SEQ ID NO: 326 - RNA, 20 nt, Artificial Sequence
  source: /note="Description of Artificial Sequence: Synthetic oligonucleotide"
gcgcugucgguugaugugau

SEQ ID NO: 327 - RNA, 20 nt, Artificial Sequence
  source: /note="Description of Artificial Sequence: Synthetic oligonucleotide"
guaucaccgguugaugugau

SEQ ID NO: 328 - RNA, 20 nt, Artificial Sequence
  source: /note="Description of Artificial Sequence: Synthetic oligonucleotide"
gcgccaccgguugauacagc

SEQ ID NO: 329 - RNA, 20 nt, Artificial Sequence
  source: /note="Description of Artificial Sequence: Synthetic oligonucleotide"
gcgccaccgguuagcacgau

SEQ ID NO: 330 - RNA, 20 nt, Artificial Sequence
  source: /note="Description of Artificial Sequence: Synthetic oligonucleotide"
gcgccaccgaggagugugau

SEQ ID NO: 331 - RNA, 20 nt, Artificial Sequence
  source: /note="Description of Artificial Sequence: Synthetic oligonucleotide"
gcgccauuaagugaugugau

SEQ ID NO: 332 - RNA, 20 nt, Artificial Sequence
  source: /note="Description of Artificial Sequence: Synthetic oligonucleotide"
gcguuguugguugaugugau

SEQ ID NO: 333 - RNA, 20 nt, Artificial Sequence
  source: /note="Description of Artificial Sequence: Synthetic oligonucleotide"
auauuaccgguugaugugau

SEQ ID NO: 334 - RNA, 20 nt, Artificial Sequence
  source: /note="Description of Artificial Sequence: Synthetic oligonucleotide"
gucaccuccaaugacuaggg

SEQ ID NO: 335 - RNA, 20 nt, Artificial Sequence
  source: /note="Description of Artificial Sequence: Synthetic oligonucleotide"
gucaccuccaaugacuaaga

SEQ ID NO: 336 - RNA, 20 nt, Artificial Sequence
  source: /note="Description of Artificial Sequence: Synthetic oligonucleotide"
gucaccuccaaugauuagga

SEQ ID NO: 337 - RNA, 20 nt, Artificial Sequence
  source: /note="Description of Artificial Sequence: Synthetic oligonucleotide"
gucaccuccagugacuagga

SEQ ID NO: 338 - RNA, 20 nt, Artificial Sequence
  source: /note="Description of Artificial Sequence: Synthetic oligonucleotide"
gucacuuccaaugacuagga

SEQ ID NO: 339 - RNA, 20 nt, Artificial Sequence
  source: /note="Description of Artificial Sequence: Synthetic oligonucleotide"
aucaccuccaaugacuagga

SEQ ID NO: 340 - RNA, 20 nt, Artificial Sequence
  source: /note="Description of Artificial Sequence: Synthetic oligonucleotide"
gucaccuccaaugacuaggg

SEQ ID NO: 341 - RNA, 20 nt, Artificial Sequence
  source: /note="Description of Artificial Sequence: Synthetic oligonucleotide"
gucaccuccaaugaccaaga

SEQ ID NO: 342 - RNA, 20 nt, Artificial Sequence
  source: /note="Description of Artificial Sequence: Synthetic oligonucleotide"
gucaccuccaauggcuggga

SEQ ID NO: 343 - RNA, 20 nt, Artificial Sequence
  source: /note="Description of Artificial Sequence: Synthetic oligonucleotide"
gucaccuccaacgaccagga

SEQ ID NO: 344 - RNA, 20 nt, Artificial Sequence
  source: /note="Description of Artificial Sequence: Synthetic oligonucleotide"
gucaccuccgaugauuagga

SEQ ID NO: 345 - RNA, 20 nt, Artificial Sequence
  source: /note="Description of Artificial Sequence: Synthetic oligonucleotide"
gucaccuccaauggccaagg

SEQ ID NO: 346 - RNA, 20 nt, Artificial Sequence
  source: /note="Description of Artificial Sequence: Synthetic oligonucleotide"
gucaccuccaacgauuaagg

SEQ ID NO: 347 - RNA, 20 nt, Artificial Sequence
  source: /note="Description of Artificial Sequence: Synthetic oligonucleotide"
gucaccuccgauggcuaagg

SEQ ID NO: 348 - RNA, 20 nt, Artificial Sequence
  source: /note="Description of Artificial Sequence: Synthetic oligonucleotide"
gucaccuucaauaacuaagg

SEQ ID NO: 349 - RNA, 20 nt, Artificial Sequence
  source: /note="Description of Artificial Sequence: Synthetic oligonucleotide"
gucaccuccaauggccaaga

SEQ ID NO: 350 - RNA, 20 nt, Artificial Sequence
  source: /note="Description of Artificial Sequence: Synthetic oligonucleotide"
gucaccuccaguggcuggga

SEQ ID NO: 351 - RNA, 20 nt, Artificial Sequence
  source: /note="Description of Artificial Sequence: Synthetic oligonucleotide"
gucaccuucaacgaccagga

SEQ ID NO: 352 - RNA, 20 nt, Artificial Sequence
  source: /note="Description of Artificial Sequence: Synthetic oligonucleotide"
gucaucuccgaugauuagga

SEQ ID NO: 353 - RNA, 20 nt, Artificial Sequence
  source: /note="Description of Artificial Sequence: Synthetic oligonucleotide"
gccaccuucaauggcuagga

SEQ ID NO: 354 - RNA, 20 nt, Artificial Sequence
  source: /note="Description of Artificial Sequence: Synthetic oligonucleotide"
gcgccaccgguugaugugau

SEQ ID NO: 355 - RNA, 20 nt, Artificial Sequence
  source: /note="Description of Artificial Sequence: Synthetic oligonucleotide"
gcgccaccgguugauguaac

SEQ ID NO: 356 - RNA, 20 nt, Artificial Sequence
  source: /note="Description of Artificial Sequence: Synthetic oligonucleotide"
gcgccaccgguugacgugac

SEQ ID NO: 357 - RNA, 20 nt, Artificial Sequence
  source: /note="Description of Artificial Sequence: Synthetic oligonucleotide"
gcgccaccggcugaugugac

SEQ ID NO: 358 - RNA, 20 nt, Artificial Sequence
  source: /note="Description of Artificial Sequence: Synthetic oligonucleotide"
gcgccgccgguugaugugac

SEQ ID NO: 359 - RNA, 20 nt, Artificial Sequence
  source: /note="Description of Artificial Sequence: Synthetic oligonucleotide"
acgccaccgguugaugugac

SEQ ID NO: 360 - RNA, 20 nt, Artificial Sequence
  source: /note="Description of Artificial Sequence: Synthetic oligonucleotide"
gcgccaccgguugaugugau

SEQ ID NO: 361 - RNA, 20 nt, Artificial Sequence
  source: /note="Description of Artificial Sequence: Synthetic oligonucleotide"
gcgccaccgguugauauaac

SEQ ID NO: 362 - RNA, 20 nt, Artificial Sequence
  source: /note="Description of Artificial Sequence: Synthetic oligonucleotide"
gcgccaccgguuggugcgac

SEQ ID NO: 363 - RNA, 20 nt, Artificial Sequence
  source: /note="Description of Artificial Sequence: Synthetic oligonucleotide"
gcgccaccggucgauaugac

SEQ ID NO: 364 - RNA, 20 nt, Artificial Sequence
  source: /note="Description of Artificial Sequence: Synthetic oligonucleotide"
gcgccaccgauugacgugac

SEQ ID NO: 365 - RNA, 20 nt, Artificial Sequence
  source: /note="Description of Artificial Sequence: Synthetic oligonucleotide"
gcgccaccgguugguauaau

SEQ ID NO: 366 - RNA, 20 nt, Artificial Sequence
  source: /note="Description of Artificial Sequence: Synthetic oligonucleotide"
gcgccaccggucgacguaau

SEQ ID NO: 367 - RNA, 20 nt, Artificial Sequence
  source: /note="Description of Artificial Sequence: Synthetic oligonucleotide"
gcgccaccgauugguguaau

SEQ ID NO: 368 - RNA, 20 nt, Artificial Sequence
  source: /note="Description of Artificial Sequence: Synthetic oligonucleotide"
gcgccacugguuaauguaau

SEQ ID NO: 369 - RNA, 20 nt, Artificial Sequence
  source: /note="Description of Artificial Sequence: Synthetic oligonucleotide"
gcgccaccgguugguauaac

SEQ ID NO: 370 - RNA, 20 nt, Artificial Sequence
  source: /note="Description of Artificial Sequence: Synthetic oligonucleotide"
gcgccaccggcuggugcgac

SEQ ID NO: 371 - RNA, 20 nt, Artificial Sequence
  source: /note="Description of Artificial Sequence: Synthetic oligonucleotide"
gcgccacuggucgauaugac

SEQ ID NO: 372 - RNA, 20 nt, Artificial Sequence
  source: /note="Description of Artificial Sequence: Synthetic oligonucleotide"
gcgcuaccgauugacgugac

SEQ ID NO: 373 - RNA, 20 nt, Artificial Sequence
  source: /note="Description of Artificial Sequence: Synthetic oligonucleotide"
gugccacugguuggugugac

SEQ ID NO: 374 - RNA, 23 nt, Artificial Sequence
  source: /note="Description of Artificial Sequence: Synthetic oligonucleotide"
gaguccgagcagaagaagaaggg

SEQ ID NO: 375 - DNA, 23 bp, Artificial Sequence
  source: /note="Description of Artificial Sequence: Synthetic oligonucleotide"
  source: /note="Description of Combined DNA/RNA Molecule: Synthetic oligonucleotide"
gauuccuaccagaagaagaatgg

SEQ ID NO: 376 - RNA, 23 nt, Artificial Sequence
  source: /note="Description of Artificial Sequence: Synthetic oligonucleotide"
aaguccgaggagaggaagaaagg

SEQ ID NO: 377 - RNA, 23 nt, Artificial Sequence
  source: /note="Description of Artificial Sequence: Synthetic oligonucleotide"
aaguccgagaagaagcagaaaag

SEQ ID NO: 378 - RNA, 23 nt, Artificial Sequence
  source: /note="Description of Artificial Sequence: Synthetic oligonucleotide"
gaguuccagaagaagaagaagag

SEQ ID NO: 379 - RNA, 23 nt, Artificial Sequence
  source: /note="Description of Artificial Sequence: Synthetic oligonucleotide"
gagucugaacggaagaagaaaag

SEQ ID NO: 380 - RNA, 23 nt, Artificial Sequence
  source: /note="Description of Artificial Sequence: Synthetic oligonucleotide"
gaguuugaguagaagaagaagag

SEQ ID NO: 381 - RNA, 23 nt, Artificial Sequence
  source: /note="Description of Artificial Sequence: Synthetic oligonucleotide"
gagucccagaagaagaaaaaaag

SEQ ID NO: 382 - DNA, 23 bp, Artificial Sequence
  source: /note="Description of Artificial Sequence: Synthetic oligonucleotide"
  source: /note="Description of Combined DNA/RNA Molecule: Synthetic oligonucleotide"
gacuccgagcagcagaaggatgg

SEQ ID NO: 383 - RNA, 23 nt, Artificial Sequence
  source: /note="Description of Artificial Sequence: Synthetic oligonucleotide"
gagucagagcagaacuagaaggg

SEQ ID NO: 384 - RNA, 23 nt, Artificial Sequence
  source: /note="Description of Artificial Sequence: Synthetic oligonucleotide"
gaggccgagcagaagaaagacgg

SEQ ID NO: 385 - RNA, 23 nt, Artificial Sequence
  source: /note="Description of Artificial Sequence: Synthetic oligonucleotide"
gagucagaccaggagaagaagag

SEQ ID NO: 386 - DNA, 23 bp, Artificial Sequence
  source: /note="Description of Artificial Sequence: Synthetic oligonucleotide"
  source: /note="Description of Combined DNA/RNA Molecule: Synthetic oligonucleotide"
gaguccaagaagaauaagaatag

SEQ ID NO: 387 - RNA, 23 nt, Artificial Sequence
  source: /note="Description of Artificial Sequence: Synthetic oligonucleotide"
gaguaagagaagaagaagaaggg

SEQ ID NO: 388 - RNA, 23 nt, Artificial Sequence
  source: /note="Description of Artificial Sequence: Synthetic oligonucleotide"
gaguaggaggagaagaagaaagg

SEQ ID NO: 389 - DNA, 23 bp, Artificial Sequence
  source: /note="Description of Artificial Sequence: Synthetic oligonucleotide"
  source: /note="Description of Combined DNA/RNA Molecule: Synthetic oligonucleotide"
aagucugagcacaagaagaatgg

SEQ ID NO: 390 - RNA, 23 nt, Artificial Sequence
  source: /note="Description of Artificial Sequence: Synthetic oligonucleotide"
gagcccgagcagaaggaggaggg

SEQ ID NO: 391 - RNA, 23 nt, Artificial Sequence
  source: /note="Description of Artificial Sequence: Synthetic oligonucleotide"
gaguuagagcagaagaagaaagg

SEQ ID NO: 392 - RNA, 23 nt, Artificial Sequence
  source: /note="Description of Artificial Sequence: Synthetic oligonucleotide"
gagucagaacagaagaacaacag

SEQ ID NO: 393 - DNA, 23 bp, Artificial Sequence
  source: /note="Description of Artificial Sequence: Synthetic oligonucleotide"
  source: /note="Description of Combined DNA/RNA Molecule: Synthetic oligonucleotide"
acgucugagcagaagaagaatgg

SEQ ID NO: 394 - RNA, 23 nt, Artificial Sequence
  source: /note="Description of Artificial Sequence: Synthetic oligonucleotide"
gaguacuagaagaagaagaaaag

SEQ ID NO: 395 - RNA, 23 nt, Artificial Sequence
  source: /note="Description of Artificial Sequence: Synthetic oligonucleotide"
aagucugagcagaagaagcacag

SEQ ID NO: 396 - RNA, 23 nt, Artificial Sequence
  source: /note="Description of Artificial Sequence: Synthetic oligonucleotide"
gagucccagcagaggaagcagag

SEQ ID NO: 397 - RNA, 23 nt, Artificial Sequence
  source: /note="Description of Artificial Sequence: Synthetic oligonucleotide"
gagucugggcaggagaagaagag

SEQ ID NO: 398 - RNA, 23 nt, Artificial Sequence
  source: /note="Description of Artificial Sequence: Synthetic oligonucleotide"
gaguccuagcaggagaagaagag

SEQ ID NO: 399 - RNA, 23 nt, Artificial Sequence
  source: /note="Description of Artificial Sequence: Synthetic oligonucleotide"
gaggaggagcagaagaagaaaag

SEQ ID NO: 400 - RNA, 23 nt, Artificial Sequence
  source: /note="Description of Artificial Sequence: Synthetic oligonucleotide"
gaguccgagaaaaugaagaagag

SEQ ID NO: 401 - RNA, 23 nt, Artificial Sequence
  source: /note="Description of Artificial Sequence: Synthetic oligonucleotide"
gaggcccagcagaggaagaagag

SEQ ID NO: 402 - RNA, 23 nt, Artificial Sequence
  source: /note="Description of Artificial Sequence: Synthetic oligonucleotide"
gaauccaagcagaagaagagaag

SEQ ID NO: 403 - DNA, 23 bp, Artificial Sequence
  source: /note="Description of Artificial Sequence: Synthetic oligonucleotide"
  source: /note="Description of Combined DNA/RNA Molecule: Synthetic oligonucleotide"
gacuccuagcaaaagaagaatgg

SEQ ID NO: 404 - RNA, 23 nt, Artificial Sequence
  source: /note="Description of Artificial Sequence: Synthetic oligonucleotide"
gagucccagcaaaagaagaaaag

SEQ ID NO: 405 - RNA, 23 nt, Artificial Sequence
  source: /note="Description of Artificial Sequence: Synthetic oligonucleotide"
gagucuaagcagaagaagaagag

SEQ ID NO: 406 - RNA, 23 nt, Artificial Sequence
  source: /note="Description of Artificial Sequence: Synthetic oligonucleotide"
aagucagaggagaagaagaaggg

SEQ ID NO: 407 - DNA, 23 bp, Artificial Sequence
  source: /note="Description of Artificial Sequence: Synthetic oligonucleotide"
  source: /note="Description of Combined DNA/RNA Molecule: Synthetic oligonucleotide"
gaguccaagcagaagaaggatag

SEQ ID NO: 408 - RNA, 23 nt, Artificial Sequence
  source: /note="Description of Artificial Sequence: Synthetic oligonucleotide"
gagacugagaagaagaagaaagg

SEQ ID NO: 409 - RNA, 23 nt, Artificial Sequence
  source: /note="Description of Artificial Sequence: Synthetic oligonucleotide"
gagucccaggagaagaagagagg

SEQ ID NO: 410 - RNA, 23 nt, Artificial Sequence
  source: /note="Description of Artificial Sequence: Synthetic oligonucleotide"
gagucccaggagaagaaaaacag

SEQ ID NO: 411 - RNA, 23 nt, Artificial Sequence
  source: /note="Description of Artificial Sequence: Synthetic oligonucleotide"
gagagcaagcagaagaagaaaag

SEQ ID NO: 412 - RNA, 23 nt, Artificial Sequence
  source: /note="Description of Artificial Sequence: Synthetic oligonucleotide"
gaguccaagcauaagaaaaacag

SEQ ID NO: 413 - RNA, 23 nt, Artificial Sequence
  source: /note="Description of Artificial Sequence: Synthetic oligonucleotide"
gaguccaagcaguagaggaaggg

SEQ ID NO: 414 - RNA, 23 nt, Artificial Sequence
  source: /note="Description of Artificial Sequence: Synthetic oligonucleotide"
gaguccgggaaggagaagaaagg

SEQ ID NO: 415 - RNA, 20 nt, Artificial Sequence
  source: /note="Description of Artificial Sequence: Synthetic oligonucleotide"
gcgccaccgguugaugugau

SEQ ID NO: 416 - RNA, 23 nt, Artificial Sequence
  source: /note="Description of Artificial Sequence: Synthetic oligonucleotide"
gggccauggguugaugugaugag

SEQ ID NO: 417 - DNA, 23 bp, Artificial Sequence
  source: /note="Description of Artificial Sequence: Synthetic oligonucleotide"
  source: /note="Description of Combined DNA/RNA Molecule: Synthetic oligonucleotide"
gtcacctccaatgactagggtgg

SEQ ID NO: 418 - DNA, 23 bp, Artificial Sequence
  source: /note="Description of Artificial Sequence: Synthetic oligonucleotide"
  source: /note="Description of Combined DNA/RNA Molecule: Synthetic oligonucleotide"
gcuacctccagtgactagggagg

SEQ ID NO: 419 - DNA, 23 bp, Artificial Sequence
  source: /note="Description of Artificial Sequence: Synthetic oligonucleotide"
  source: /note="Description of Combined DNA/RNA Molecule: Synthetic oligonucleotide"
gtgacctccaatgcctagagggg

SEQ ID NO: 420 - DNA, 23 bp, Artificial Sequence
  source: /note="Description of Artificial Sequence: Synthetic oligonucleotide"
  source: /note="Description of Combined DNA/RNA Molecule: Synthetic oligonucleotide"
gtcacctccactucctagggcag

SEQ ID NO: 421 - DNA, 23 bp, Artificial Sequence
  source: /note="Description of Artificial Sequence: Synthetic oligonucleotide"
  source: /note="Description of Combined DNA/RNA Molecule: Synthetic oligonucleotide"
utcacctccaaaaactagggaag

SEQ ID NO: 422 - DNA, 23 bp, Artificial Sequence
  source: /note="Description of Artificial Sequence: Synthetic oligonucleotide"
  source: /note="Description of Combined DNA/RNA Molecule: Synthetic oligonucleotide"
gtcaactccaatggctugggagg

SEQ ID NO: 423 - DNA, 23 bp, Artificial Sequence
  source: /note="Description of Artificial Sequence: Synthetic oligonucleotide"
  source: /note="Description of Combined DNA/RNA Molecule: Synthetic oligonucleotide"
gtcacctuaaatgactugggaag

SEQ ID NO: 424 - DNA, 23 bp, Artificial Sequence
  source: /note="Description of Artificial Sequence: Synthetic oligonucleotide"
  source: /note="Description of Combined DNA/RNA Molecule: Synthetic oligonucleotide"
gtcacutccaaggactagagaag

SEQ ID NO: 425 - DNA, 23 bp, Artificial Sequence
  source: /note="Description of Artificial Sequence: Synthetic oligonucleotide"
  source: /note="Description of Combined DNA/RNA Molecule: Synthetic oligonucleotide"
gtcacctccaggguctagggcag

SEQ ID NO: 426 - DNA, 23 bp, Artificial Sequence
  source: /note="Description of Artificial Sequence: Synthetic oligonucleotide"
  source: /note="Description of Combined DNA/RNA Molecule: Synthetic oligonucleotide"
gtcacctccactguatagggagg

SEQ ID NO: 427 - DNA, 23 bp, Artificial Sequence
  source: /note="Description of Artificial Sequence: Synthetic oligonucleotide"
  source: /note="Description of Combined DNA/RNA Molecule: Synthetic oligonucleotide"
gtcaactccaatgautaggacag

SEQ ID NO: 428 - DNA, 23 bp, Artificial Sequence
  source: /note="Description of Artificial Sequence: Synthetic oligonucleotide"
gtggtgtcacgctcgtcgtttgg

SEQ ID NO: 429 - DNA, 23 bp, Artificial Sequence
  source: /note="Description of Artificial Sequence: Synthetic oligonucleotide"
tccagtctattaattgttgccgg

SEQ ID NO: 430 - DNA, 12 bp, Homo sapiens
tagcgggtaagc

SEQ ID NO: 431 - DNA, 12 bp, Homo sapiens
tcggtcacatgt

SEQ ID NO: 432 - DNA, 12 bp, Homo sapiens
actccccgtagg

SEQ ID NO: 433 - DNA, 12 bp, Homo sapiens
actgcgtgttaa

SEQ ID NO: 434 - DNA, 12 bp, Homo sapiens
acgtcgcctgat

SEQ ID NO: 435 - DNA, 12 bp, Homo sapiens
taggtcgaccag

SEQ ID NO: 436 - DNA, 12 bp, Homo sapiens
ggcgttaatgat

SEQ ID NO: 437 - DNA, 12 bp, Homo sapiens
tgtcgcatgtta

SEQ ID NO: 438 - DNA, 12 bp, Homo sapiens
atggaaacgcat

SEQ ID NO: 439 - DNA, 12 bp, Homo sapiens
gccgaattcctc

SEQ ID NO: 440 - DNA, 12 bp, Homo sapiens
gcatggtacgga

SEQ ID NO: 441 - DNA, 12 bp, Homo sapiens
cggtactcttac

SEQ ID NO: 442 - DNA, 12 bp, Homo sapiens
gcctgtgccgta

SEQ ID NO: 443 - DNA, 12 bp, Homo sapiens
tacggtaagtcg

SEQ ID NO: 444 - DNA, 12 bp, Homo sapiens
cacgaaattacc

SEQ ID NO: 445 - DNA, 12 bp, Homo sapiens
aaccaagatacg

SEQ ID NO: 446 - DNA, 12 bp, Homo sapiens
gagtcgatacgc

SEQ ID NO: 447 - DNA, 12 bp, Homo sapiens
gtctcacgatcg

SEQ ID NO: 448 - DNA, 12 bp, Homo sapiens
tcgtcgggtgca

SEQ ID NO: 449 - DNA, 12 bp, Homo sapiens
actccgtagtga

SEQ ID NO: 450 - DNA, 12 bp, Homo sapiens
caggacgtccgt

SEQ ID NO: 451 - DNA, 12 bp, Homo sapiens
tcgtatccctac

SEQ ID NO: 452 - DNA, 12 bp, Homo sapiens
tttcaaggccgg

SEQ ID NO: 453 - DNA, 12 bp, Homo sapiens
cgccggtggaat

SEQ ID NO: 454 - DNA, 12 bp, Homo sapiens
gaacccgtccta

SEQ ID NO: 455 - DNA, 12 bp, Homo sapiens
gattcatcagcg

SEQ ID NO: 456 - DNA, 12 bp, Homo sapiens
acaccggtcttc

SEQ ID NO: 457 - DNA, 12 bp, Homo sapiens
atcgtgccctaa

SEQ ID NO: 458 - DNA, 12 bp, Homo sapiens
gcgtcaatgttc

SEQ ID NO: 459 - DNA, 12 bp, Homo sapiens
ctccgtatctcg

SEQ ID NO: 460 - DNA, 12 bp, Homo sapiens
ccgattccttcg

SEQ ID NO: 461 - DNA, 12 bp, Homo sapiens
tgcgcctccagt

SEQ ID NO: 462 - DNA, 12 bp, Homo sapiens
taacgtcggagc

SEQ ID NO: 463 - DNA, 12 bp, Homo sapiens
aaggtcgcccat

SEQ ID NO: 464 - DNA, 12 bp, Homo sapiens
ctcggggactat

SEQ ID NO: 465 - DNA, 12 bp, Homo sapiens
ttcgagcgattt

SEQ ID NO: 466 - DNA, 12 bp, Homo sapiens
tgagtcgtcgag

SEQ ID NO: 467 - DNA, 12 bp, Homo sapiens
tttacgcagagg

SEQ ID NO: 468 - DNA, 12 bp, Homo sapiens
aggaagtatcgc

SEQ ID NO: 469 - DNA, 12 bp, Homo sapiens
actcgataccat

SEQ ID NO: 470 - DNA, 12 bp, Homo sapiens
cgctacatagca

SEQ ID NO: 471 - DNA, 12 bp, Homo sapiens
ttcataaccggc

SEQ ID NO: 472 - DNA, 12 bp, Homo sapiens
ccaaacggttaa

SEQ ID NO: 473 - DNA, 12 bp, Homo sapiens
cgattccttcgt

SEQ ID NO: 474 - DNA, 12 bp, Homo sapiens
cgtcatgaataa

SEQ ID NO: 475 - DNA, 12 bp, Homo sapiens
agtggcgatgac

SEQ ID NO: 476 - DNA, 12 bp, Homo sapiens
cccctacggcac

SEQ ID NO: 477 - DNA, 12 bp, Homo sapiens
gccaacccgcac

SEQ ID NO: 478 - DNA, 12 bp, Homo sapiens
tgggacaccggt

SEQ ID NO: 479 - DNA, 12 bp, Homo sapiens
ttgactgcggcg

SEQ ID NO: 480 - DNA, 12 bp, Homo sapiens
actatgcgtagg

SEQ ID NO: 481 - DNA, 12 bp, Homo sapiens
tcacccaaagcg

SEQ ID NO: 482 - DNA, 12 bp, Homo sapiens
gcaggacgtccg

SEQ ID NO: 483 - DNA, 12 bp, Homo sapiens
acaccgaaaacg

SEQ ID NO: 484 - DNA, 12 bp, Homo sapiens
cggtgtattgag

SEQ ID NO: 485 - DNA, 12 bp, Homo sapiens
cacgaggtatgc

SEQ ID NO: 486 - DNA, 12 bp, Homo sapiens
taaagcgacccg

SEQ ID NO: 487 - DNA, 12 bp, Homo sapiens
cttagtcggcca

SEQ ID NO: 488 - DNA, 12 bp, Homo sapiens
cgaaaacgtggc

SEQ ID NO: 489 - DNA, 12 bp, Homo sapiens
cgtgccctgaac

SEQ ID NO: 490 - DNA, 12 bp, Homo sapiens
tttaccatcgaa

SEQ ID NO: 491 - DNA, 12 bp, Homo sapiens
cgtagccatgtt

SEQ ID NO: 492 - DNA, 12 bp, Homo sapiens
cccaaacggtta

SEQ ID NO: 493 - DNA, 12 bp, Homo sapiens
gcgttatcagaa

SEQ ID NO: 494 - DNA, 12 bp, Homo sapiens
tcgatggtaaac

SEQ ID NO: 495 - DNA, 12 bp, Homo sapiens
cgactttttgca

SEQ ID NO: 496 - DNA, 12 bp, Homo sapiens
tcgacgactcac

SEQ ID NO: 497 - DNA, 12 bp, Homo sapiens
acgcgtcagata

SEQ ID NO: 498 - DNA, 12 bp, Homo sapiens
cgtacggcacag

SEQ ID NO: 499 - DNA, 12 bp, Homo sapiens
ctatgccgtgca

SEQ ID NO: 500 - DNA, 12 bp, Homo sapiens
cgcgtcagatat

SEQ ID NO: 501 - DNA, 12 bp, Homo sapiens
aagatcggtagc

SEQ ID NO: 502 - DNA, 12 bp, Homo sapiens
cttcgcaaggag

SEQ ID NO: 503 - DNA, 12 bp, Homo sapiens
gtcgtggactac

SEQ ID NO: 504 - DNA, 12 bp, Homo sapiens
ggtcgtcatcaa

SEQ ID NO: 505 - DNA, 12 bp, Homo sapiens
gttaacagcgtg

SEQ ID NO: 506 - DNA, 12 bp, Homo sapiens
tagctaaccgtt

SEQ ID NO: 507 - DNA, 12 bp, Homo sapiens
agtaaaggcgct

SEQ ID NO: 508 - DNA, 12 bp, Homo sapiens
ggtaatttcgtg

SEQ ID NO: 509 - DNA, 20 bp, Mus musculus
gactgattcagctagaccgg

SEQ ID NO: 510 - DNA, 20 bp, Mus musculus
ggcacaaacgcgttcaatac

SEQ ID NO: 511 - DNA, 20 bp, Mus musculus
aacgcgttcaataccggtct

SEQ ID NO: 512 - DNA, 20 bp, Rattus norvegicus
gctaggaggatctcgggcgg

SEQ ID NO: 513 - DNA, 20 bp, Rattus norvegicus
gttccagcccgcgactaagc

SEQ ID NO: 514 - DNA, 20 bp, Rattus norvegicus
gtgagggggttgcaacgagg

SEQ ID NO: 515 - DNA, 20 bp, Rattus norvegicus
accgcaactcttggcgcgtc

SEQ ID NO: 516 - DNA, 20 bp, Rattus norvegicus
accagatgcggttgcagtcg

SEQ ID NO: 517 - DNA, 20 bp, Rattus norvegicus
tacttcggcgcgtattttta

SEQ ID NO: 518 - DNA, 20 bp, Rattus norvegicus
aaatgtgagattccggacta

SEQ ID NO: 519 - DNA, 20 bp, Rattus norvegicus
tgtgaccgcgcttgcgaact

SEQ ID NO: 520 - DNA, 20 bp, Rattus norvegicus
tctcgggcaccgcgagccgg

SEQ ID NO: 521 - DNA, 20 bp, Rattus norvegicus
cgctcctggctggtccgcaa

SEQ ID NO: 522 - DNA, 20 bp, Rattus norvegicus
tgagggtagttgagcgccgt

SEQ ID NO: 523 - DNA, 20 bp, Rattus norvegicus
tgagattgggaccgccacgc

SEQ ID NO: 524 - DNA, 20 bp, Rattus norvegicus
ttgatatagactttacgtgc

SEQ ID NO: 525 - DNA, 20 bp, Rattus norvegicus
agctaactacccccccgggt

SEQ ID NO: 526 - DNA, 20 bp, Rattus norvegicus
cacctccagcatcgggcgag

SEQ ID NO: 527 - DNA, 20 bp, Rattus norvegicus
aggcggcgtcgtcgggatgt

SEQ ID NO: 528 - DNA, 20 bp, Rattus norvegicus
ccgtttggcccccagttcgg

SEQ ID NO: 529 - DNA, 20 bp, Rattus norvegicus
ttccagcccgcgactaagcg

SEQ ID NO: 530 - DNA, 20 bp, Rattus norvegicus
agagtgagggggttgcaacg

SEQ ID NO: 531 - DNA, 20 bp, Rattus norvegicus
ccgcaactcttggcgcgtcg

SEQ ID NO: 532 - DNA, 20 bp, Rattus norvegicus
tgatcccgctcgcccgatgc

SEQ ID NO: 533 - DNA, 20 bp, Rattus norvegicus
ctggaagaggcggcgtcgtc

SEQ ID NO: 534 - DNA, 20 bp, Rattus norvegicus
aaccccgcttagtcgcgggc

SEQ ID NO: 535 - DNA, 20 bp, Rattus norvegicus
attgggaccgccacgccggt

SEQ ID NO: 536 - DNA, 20 bp, Rattus norvegicus
tccagaaccgcgtctcgacg

SEQ ID NO: 537 - DNA, 20 bp, Rattus norvegicus
cgcgcacagaacgcgtacgc

SEQ ID NO: 538 - DNA, 20 bp, Rattus norvegicus
gtgaaaccccgcttagtcgc

SEQ ID NO: 539 - DNA, 20 bp, Rattus norvegicus
ccccgacgcgccaagagttg

SEQ ID NO: 540 - DNA, 20 bp, Rattus norvegicus
accgcgtctcgacgcggaga

SEQ ID NO: 541 - DNA, 20 bp, Rattus norvegicus
ccgcgcacagaacgcgtacg

SEQ ID NO: 542 - DNA, 20 bp, Rattus norvegicus
ggtgaaaccccgcttagtcg

SEQ ID NO: 543 - DNA, 20 bp, Rattus norvegicus
actcttggcgcgtcggggca

SEQ ID NO: 544 - DNA, 20 bp, Rattus norvegicus
tccttctccgcgtcgagacg

SEQ ID NO: 545 - DNA, 20 bp, Rattus norvegicus
acggtccggacctccgaact

SEQ ID NO: 546 - DNA, 20 bp, Rattus norvegicus
ggcgccagccgctcgctcta

SEQ ID NO: 547 - DNA, 20 bp, Rattus norvegicus
gacttccgagttcgcaagcg

SEQ ID NO: 548 - DNA, 20 bp, Rattus norvegicus
tgcgaactcggaagtccaat

SEQ ID NO: 549 - DNA, 20 bp, Rattus norvegicus
tctggaagaggcggcgtcgt

SEQ ID NO: 550 - DNA, 20 bp, Rattus norvegicus
tcttagccccgagacccggt

SEQ ID NO: 551 - DNA, 20 bp, Rattus norvegicus
ccctccggcgccgtgttttc

SEQ ID NO: 552 - DNA, 20 bp, Rattus norvegicus
ccagaaaacacggcgccgga

SEQ ID NO: 553 - DNA, 17 bp, Danio rerio
atcaatatctcgcccag

SEQ ID NO: 554 - DNA, 17 bp, Danio rerio
attaaacgtgttccact

SEQ ID NO: 555 - DNA, 17 bp, Danio rerio
acgtttaatcgctttct

SEQ ID NO: 556 - DNA, 17 bp, Danio rerio
caagatgcgtacggtca

SEQ ID NO: 557 - DNA, 17 bp, Danio rerio
tctgtgtactcgaatat

SEQ ID NO: 558 - DNA, 17 bp, Danio rerio
tcctgacttctgggcac

SEQ ID NO: 559 - DNA, 17 bp, Danio rerio
cccggtgcccagaagtc

SEQ ID NO: 560 - DNA, 17 bp, Danio rerio
ccggagatccattcatg

SEQ ID NO: 561 - DNA, 17 bp, Danio rerio
tgatgacccagaatcaa

SEQ ID NO: 562 - DNA, 17 bp, Danio rerio
tgaatgaccggtcctcc

SEQ ID NO: 563 - DNA, 17 bp, Danio rerio
tccaaaggggcttcgga

SEQ ID NO: 564 - DNA, 17 bp, Danio rerio
cttcagttcgctgtgca

SEQ ID NO: 565 - DNA, 17 bp, Danio rerio
gatacacgccggcataa

SEQ ID NO: 566 - DNA, 17 bp, Danio rerio
cacacgaggatacacgc

SEQ ID NO: 567 - DNA, 17 bp, Danio rerio
tcgctgtcctcttcact

SEQ ID NO: 568 - DNA, 17 bp, Danio rerio
ttaaagtgattcccagt

SEQ ID NO: 569 - DNA, 17 bp, Danio rerio
cagctgatcctccaact

SEQ ID NO: 570 - DNA, 17 bp, Danio rerio
atatttagagtaagaat

SEQ ID NO: 571 - DNA, 17 bp, Drosophila melanogaster
aatttttatcattcagt

SEQ ID NO: 572 - DNA, 20 bp, Drosophila melanogaster
gattcttccatgatcggcca

SEQ ID NO: 573 - DNA, 20 bp, Drosophila melanogaster
cgattgaaaatccacataaa

SEQ ID NO: 574 - DNA, 20 bp, Drosophila melanogaster
gctgatttcggacaaaagtc

SEQ ID NO: 575 - DNA, 20 bp, Drosophila melanogaster
aaacggatgacgtgcaacgt

SEQ ID NO: 576 - DNA, 20 bp, Drosophila melanogaster
cgttttgtgtgcgtgcgcac

SEQ ID NO: 577 - DNA, 20 bp, Drosophila melanogaster
ggaataatcttcgtctatcc

SEQ ID NO: 578 - DNA, 20 bp, Drosophila melanogaster
ttcgctcacgaacaccaaca

SEQ ID NO: 579 - DNA, 20 bp, Drosophila melanogaster
acaaagtacatagggtgttt

SEQ ID NO: 580 - DNA, 20 bp, Drosophila melanogaster
ccatcccccgtaaagagggt

SEQ ID NO: 581 - DNA, 20 bp, Drosophila melanogaster
tatttttagttggtaaatta

SEQ ID NO: 582 - DNA, 17 bp, Drosophila melanogaster
attcactctgggttatg

SEQ ID NO: 583 - DNA, 20 bp, Drosophila melanogaster
ctgctttccttggccgatca

SEQ ID NO: 584 - DNA, 20 bp, Drosophila melanogaster
gattatttgctccatttatg

SEQ ID NO: 585 - DNA, 20 bp, Drosophila melanogaster
ctctgtacagaatattttct

SEQ ID NO: 586 - DNA, 20 bp, Drosophila melanogaster
gcagcggcagtgagagacgt

SEQ ID NO: 587 - DNA, 20 bp, Drosophila melanogaster
tgtgcgcacgcacacaaaac

SEQ ID NO: 588 - DNA, 20 bp, Drosophila melanogaster
aattcgctaattgggcagcc

SEQ ID NO: 589 - DNA, 20 bp, Drosophila melanogaster
caaggaaattgacagatgta

SEQ ID NO: 590 - DNA, 20 bp, Drosophila melanogaster
gctctagcaaccacgtcaga

SEQ ID NO: 591 - DNA, 20 bp, Drosophila melanogaster
acaatacgaatgcgagaagg

SEQ ID NO: 592 - DNA, 20 bp, Drosophila melanogaster
aaataaaaattagtgtccgc

SEQ ID NO: 593 - DNA, 17 bp, Drosophila melanogaster
agagtgaataaattaca

SEQ ID NO: 594 - DNA, 20 bp, Drosophila melanogaster
ttattcaagacttacaccat

SEQ ID NO: 595 - DNA, 20 bp, Drosophila melanogaster
attatgacgttttttggtac

SEQ ID NO: 596 - DNA, 20 bp, Drosophila melanogaster
ttcgggcggtctaaagcagt

SEQ ID NO: 597 - DNA, 20 bp, Drosophila melanogaster
tgttactttttcgaacgttg

SEQ ID NO: 598 - DNA, 20 bp, Drosophila melanogaster
gttttgtgtgcgtgcgcaca

SEQ ID NO: 599 - DNA, 20 bp, Drosophila melanogaster
tgcccaattagcgaattagg

SEQ ID NO: 600 - DNA, 20 bp, Drosophila melanogaster
cgccccaaaagaaaatacgt

SEQ ID NO: 601 - DNA, 20 bp, Drosophila melanogaster
gctgcggctttcgtgaaatg

SEQ ID NO: 602 - DNA, 20 bp, Drosophila melanogaster
aaaaggaggagaacatatct

SEQ ID NO: 603 - DNA, 17 bp, Drosophila melanogaster
atgtaatttattcactc

SEQ ID NO: 604 - DNA, 20 bp, Drosophila melanogaster
agaactaagcacgtattttt

SEQ ID NO: 605 - DNA, 20 bp, Drosophila melanogaster
acaaacaatccaaataaaag

SEQ ID NO: 606 - DNA, 20 bp, Drosophila melanogaster
caacaaaaaagtgagctctg

SEQ ID NO: 607 - DNA, 20 bp, Drosophila melanogaster
cgttgttcgtttttgtagtt

SEQ ID NO: 608 - DNA, 20 bp, Drosophila melanogaster
ctctttctggtaaatgctgt

SEQ ID NO: 609 - DNA, 20 bp, Drosophila melanogaster
ttaggtgggattttcgtgta

SEQ ID NO: 610 - DNA, 20 bp, Drosophila melanogaster
ctacaaaactacacgaatta

SEQ ID NO: 611 - DNA, 20 bp, Drosophila melanogaster
gctctcgctctgcctcgctg

SEQ ID NO: 612 - DNA, 20 bp, Drosophila melanogaster
aaaggaggagaacatatctt

SEQ ID NO: 613 - DNA, 17 bp, Drosophila melanogaster
aatcaaatcggtacatt

SEQ ID NO: 614 - DNA, 20 bp, Drosophila melanogaster
atttcagctctcaacgcaaa

SEQ ID NO: 615 - DNA, 20 bp, Drosophila melanogaster
attctgaaaccacttttatt

SEQ ID NO: 616 - DNA, 20 bp, Drosophila melanogaster
gagctctgcggtagtgacgc

SEQ ID NO: 617 - DNA, 20 bp, Drosophila melanogaster
ctacaaaaacgaacaacgca

SEQ ID NO: 618 - DNA, 20 bp, Drosophila melanogaster
tactaaacacatactaaaac

SEQ ID NO: 619 - DNA, 20 bp, Drosophila melanogaster
gtcgatttgtagaactggtg

SEQ ID NO: 620 - DNA, 20 bp, Drosophila melanogaster
tggtacttttctctcgtaca

SEQ ID NO: 621 - DNA, 20 bp, Drosophila melanogaster
ttccatgcttctttagtgca

SEQ ID NO: 622 - DNA, 20 bp, Drosophila melanogaster
attaaaagcgtatttttagt

SEQ ID NO: 623 - DNA, 17 bp, Drosophila melanogaster
ggttcgacacgcagaaa

SEQ ID NO: 624 - DNA, 20 bp, Drosophila melanogaster
tggagcaaataatccattca

SEQ ID NO: 625 - DNA, 20 bp, Drosophila melanogaster
gctctgtacagaatattttc

SEQ ID NO: 626 - DNA, 20 bp, Drosophila melanogaster
atgttactttttcgaacgtt

SEQ ID NO: 627 - DNA, 20 bp, Drosophila melanogaster
atcccgttagtgtgtgagat

SEQ ID NO: 628 - DNA, 20 bp, Drosophila melanogaster
taggtgggattttcgtgtag

SEQ ID NO: 629 - DNA, 20 bp, Drosophila melanogaster
tctttatgtacacgagtata

SEQ ID NO: 630 - DNA, 20 bp, Drosophila melanogaster
ttccatgcactaaagaagca

SEQ ID NO: 631 - DNA, 20 bp, Drosophila melanogaster
ggtcgcgtcgataccatttt

SEQ ID NO: 632 - DNA, 20 bp, Drosophila melanogaster
ctttcttcctcttcttcggg

SEQ ID NO: 633 - DNA, 20 bp, Drosophila melanogaster
catgttactttttcgaacgt

SEQ ID NO: 634 - DNA, 20 bp, Drosophila melanogaster
tccccaatctcacacactaa

SEQ ID NO: 635 - DNA, 20 bp, Drosophila melanogaster
tgtaggggtccctatagtag

SEQ ID NO: 636 - DNA, 20 bp, Drosophila melanogaster
cacaaagtacatagggtgtt

SEQ ID NO: 637 - DNA, 20 bp, Drosophila melanogaster
tcccccatcccccgtaaaga

SEQ ID NO: 638 - DNA, 20 bp, Drosophila melanogaster
ctttagaccgcccgaagaag

SEQ ID NO: 639 - DNA, 20 bp, Drosophila melanogaster
tacaaaaacgaacaacgcaa

SEQ ID NO: 640 - DNA, 20 bp, Drosophila melanogaster
gttgaatcgcctgtctttaa

SEQ ID NO: 641 - DNA, 20 bp, Drosophila melanogaster
ccgcgctgctcatccaaact

SEQ ID NO: 642 - DNA, 20 bp, Drosophila melanogaster
cttcagcgcacaaagtacat

SEQ ID NO: 643 - DNA, 20 bp, Drosophila melanogaster
gcaacaatacgaatgcgaga

SEQ ID NO: 644 - DNA, 20 bp, Drosophila melanogaster
gccggcagaggcagtgaccg

SEQ ID NO: 645 - DNA, 20 bp, Drosophila melanogaster
cgcaagggagcaatgggtac

SEQ ID NO: 646 - DNA, 20 bp, Drosophila melanogaster
ttgaatcgcctgtctttaat

SEQ ID NO: 647 - DNA, 20 bp, Drosophila melanogaster
agaaactttcacggcaccgt

SEQ ID NO: 648 - DNA, 20 bp, Drosophila melanogaster
gcaagcgaaatggcgcttcg

SEQ ID NO: 649 - DNA, 20 bp, Drosophila melanogaster
agaggcagtgaccgaggcag

SEQ ID NO: 650 - DNA, 20 bp, Drosophila melanogaster
ggaaaaaacccattaaagac

SEQ ID NO: 651 - DNA, 20 bp, Drosophila melanogaster
atgcacggaataagctccaa

SEQ ID NO: 652 - DNA, 20 bp, Drosophila melanogaster
tgtaccaccaaccctcttta

SEQ ID NO: 653 - DNA, 20 bp, Drosophila melanogaster
gaaatcttcattccctccaa

SEQ ID NO: 654 - DNA, 20 bp, Drosophila melanogaster
aaggaaattgacagatgtat

SEQ ID NO: 655 - DNA, 20 bp, Drosophila melanogaster
gtaccaccaaccctctttac

SEQ ID NO: 656 - DNA, 20 bp, Drosophila melanogaster
cgcaaaaagcctctactata

SEQ ID NO: 657 - DNA, 20 bp, Drosophila melanogaster
taccaccaaccctctttacg

SEQ ID NO: 658 - DNA, 20 bp, Drosophila melanogaster
tcgcaaaaagcctctactat

SEQ ID NO: 659 - DNA, 20 bp, Drosophila melanogaster
accaccaaccctctttacgg

SEQ ID NO: 660 - DNA, 20 bp, Drosophila melanogaster
ccaaccctctttacggggga

SEQ ID NO: 661 - DNA, 20 bp, Drosophila melanogaster
caaccctctttacgggggat

SEQ ID NO: 662 - DNA, 20 bp, Drosophila melanogaster
atcccccatcccccgtaaag

SEQ ID NO: 663 - DNA, 17 bp, Caenorhabditis elegans
aagagagtcagattgga

SEQ ID NO: 664 - DNA, 17 bp, Caenorhabditis elegans
tctgactctcttgtgtt

SEQ ID NO: 665 - DNA, 17 bp, Caenorhabditis elegans
acacaagagagtcagat

SEQ ID NO: 666 - DNA, 17 bp, Caenorhabditis elegans
attttcaggtaaaagtt

SEQ ID NO: 667 - DNA, 17 bp, Caenorhabditis elegans
gaagacgctcgaattct

SEQ ID NO: 668 - DNA, 17 bp, Caenorhabditis elegans
tatgtgacgtcttatct

SEQ ID NO: 669 - DNA, 17 bp, Caenorhabditis elegans
tgttcctcttgatcatc

SEQ ID NO: 670 - DNA, 17 bp, Caenorhabditis elegans
aagaggaacataatcta

SEQ ID NO: 671 - DNA, 17 bp, Caenorhabditis elegans
tctaggccacgtcttgc

SEQ ID NO: 672 - DNA, 17 bp, Caenorhabditis elegans
agtattctatattcagt

SEQ ID NO: 673 - DNA, 17 bp, Caenorhabditis elegans
tgcatggtttgaatctt

SEQ ID NO: 674 - DNA, 17 bp, Caenorhabditis elegans
gcaactgatgtgtttct

SEQ ID NO: 675 - DNA, 17 bp, Caenorhabditis elegans
gatgtgtttctaggctc

SEQ ID NO: 676 - DNA, 17 bp, Caenorhabditis elegans
aagttctagatcacgag

SEQ ID NO: 677 - DNA, 17 bp, Caenorhabditis elegans
tcccaaatcatccttga

SEQ ID NO: 678 - DNA, 17 bp, Caenorhabditis elegans
tgggttttaaaccatca

SEQ ID NO: 679 - DNA, 17 bp, Caenorhabditis elegans
gacgggttggaggcaga

SEQ ID NO: 680 - DNA, 17 bp, Caenorhabditis elegans
cctccaacccgtccaat

SEQ ID NO: 681 - DNA, 17 bp, Caenorhabditis elegans
aaaccgattggacgggt

SEQ ID NO: 682 - DNA, 17 bp, Caenorhabditis elegans
ttggaaaccgattggac

SEQ ID NO: 683 - DNA, 17 bp, Caenorhabditis elegans
tgtctattgtacaagct

SEQ ID NO: 684 - DNA, 17 bp, Caenorhabditis elegans
gtctattgtacaagctt

SEQ ID NO: 685 - DNA, 17 bp, Caenorhabditis elegans
tctattgtacaagcttg

SEQ ID NO: 686 - DNA, 17 bp, Caenorhabditis elegans
tagcactcgacccgaaa

SEQ ID NO: 687 - DNA, 17 bp, Caenorhabditis elegans
cactcgacccgaaacgg

SEQ ID NO: 688 - DNA, 17 bp, Caenorhabditis elegans
actcgacccgaaacggt

SEQ ID NO: 689 - DNA, 16 bp, Caenorhabditis elegans
acccgaaacggtggga

SEQ ID NO: 690 - DNA, 17 bp, Caenorhabditis elegans
cccgaaacggtgggaag

SEQ ID NO: 691 - DNA, 17 bp, Caenorhabditis elegans
ccgaaacggtgggaagg

SEQ ID NO: 692 - DNA, 17 bp, Caenorhabditis elegans
aacggtgggaagggggg

SEQ ID NO: 693 - DNA, 17 bp, Caenorhabditis elegans
ccccttcccaccgtttc

SEQ ID NO: 694 - DNA, 17 bp, Caenorhabditis elegans
cccccttcccaccgttt

SEQ ID NO: 695 - DNA, 17 bp, Caenorhabditis elegans
ggggggaggacatccgc

SEQ ID NO: 696 - DNA, 17 bp, Caenorhabditis elegans
taggtgactgactccgg

SEQ ID NO: 697 - DNA, 17 bp, Caenorhabditis elegans
ttgtaggtgactgactc

SEQ ID NO: 698 - DNA, 17 bp, Caenorhabditis elegans
ggattagctgctccaat

SEQ ID NO: 699 - DNA, 17 bp, Caenorhabditis elegans
attagctgctccaattg

SEQ ID NO: 700 - DNA, 17 bp, Caenorhabditis elegans
acttagcacaccccaat

SEQ ID NO: 701 - DNA, 17 bp, Caenorhabditis elegans
aattgtctatgtttaat

SEQ ID NO: 702 - DNA, 17 bp, Caenorhabditis elegans
taatgggtgtatcgtat

SEQ ID NO: 703 - DNA, 17 bp, Caenorhabditis elegans
agcactttttgagtggt

SEQ ID NO: 704 - DNA, 17 bp, Caenorhabditis elegans
aggaagtgagagtcact

SEQ ID NO: 705 - DNA, 17 bp, Caenorhabditis elegans
ggaagtgagagtcacta

SEQ ID NO: 706 - DNA, 17 bp, Caenorhabditis elegans
gaatggataaagccacg

SEQ ID NO: 707 - DNA, 17 bp, Caenorhabditis elegans
ccacgtggcaatcatat

SEQ ID NO: 708 - DNA, 17 bp, Caenorhabditis elegans
gtttatagtaggatttt

SEQ ID NO: 709 - DNA, 20 bp, Sus scrofa
aggatacctcaacgactacg

SEQ ID NO: 710 - DNA, 20 bp, Sus scrofa
gcgctgcccgacgtgtggca

SEQ ID NO: 711 - DNA, 20 bp, Sus scrofa
cttcaagcaatagggtcccg

SEQ ID NO: 712 - DNA, 20 bp, Sus scrofa
atgacgcatatcaaatcgca

SEQ ID NO: 713 - DNA, 20 bp, Sus scrofa
tattgctctatagtcggctt

SEQ ID NO: 714 - DNA, 20 bp, Sus scrofa
ataaccgacttagcgaattc

SEQ ID NO: 715 - DNA, 20 bp, Sus scrofa
aggctgctgaccgtattgcc

SEQ ID NO: 716 - DNA, 20 bp, Sus scrofa
ggatacctcaacgactacgc

SEQ ID NO: 717 - DNA, 20 bp, Sus scrofa
ctcagccccgtgcaggccta

SEQ ID NO: 718 - DNA, 20 bp, Sus scrofa
taggaaagcggctcggattg

SEQ ID NO: 719 - DNA, 20 bp, Sus scrofa
ggcatagacgggcgttaagt

SEQ ID NO: 720 - DNA, 20 bp, Sus scrofa
gcggtccctagacccaaccg

SEQ ID NO: 721 - DNA, 20 bp, Sus scrofa
agcccgggagtctttcgcta

SEQ ID NO: 722 - DNA, 20 bp, Sus scrofa
ctgctagtggcggccgttta

SEQ ID NO: 723 - DNA, 20 bp, Sus scrofa
gatacctcaacgactacgcg

SEQ ID NO: 724 - DNA, 20 bp, Sus scrofa
ttttcccagcaatagggtcg

SEQ ID NO: 725 - DNA, 20 bp, Sus scrofa
cgaatgcccgggtacgaggg

SEQ ID NO: 726 - DNA, 20 bp, Sus scrofa
ggaaagaaagtctgcgcgtc

SEQ ID NO: 727 - DNA, 20 bp, Sus scrofa
cgggccccgcgtagtcgttg

SEQ ID NO: 728 - DNA, 20 bp, Sus scrofa
ggtctcctcgaccctattgc

SEQ ID NO: 729 - DNA, 20 bp, Sus scrofa
tttatgaacggattgcactc

SEQ ID NO: 730 - DNA, 20 bp, Sus scrofa
gcagaggccggcgggtgtaa

SEQ ID NO: 731 - DNA, 20 bp, Sus scrofa
ggcgtcgccatcgtagacgg

SEQ ID NO: 732 - DNA, 20 bp, Sus scrofa
gtctctgcgacgcgatccag

SEQ ID NO: 733 - DNA, 20 bp, Sus scrofa
tcacccaccaaccgttcatt

SEQ ID NO: 734 - DNA, 20 bp, Sus scrofa
cgtctacgatggcgacgccg

SEQ ID NO: 735 - DNA, 20 bp, Sus scrofa
agtctctgcgacgcgatcca

SEQ ID NO: 736 - DNA, 20 bp, Sus scrofa
gtaggtgcctaatgaacggt

SEQ ID NO: 737 - DNA, 20 bp, Sus scrofa
tggctacatcaacggcgacg

SEQ ID NO: 738 - DNA, 20 bp, Sus scrofa
gagtctctgcgacgcgatcc

SEQ ID NO: 739 - DNA, 20 bp, Sus scrofa
ggggcccacggttgggtcta

SEQ ID NO: 740 - DNA, 20 bp, Sus scrofa
acctccgccgtcgccgtcgg

SEQ ID NO: 741 - DNA, 20 bp, Sus scrofa
ttggcagaggatgcgaggcg

SEQ ID NO: 742 - DNA, 20 bp, Sus scrofa
cccgggccctgagcgcgcct

SEQ ID NO: 743 - DNA, 20 bp, Sus scrofa
cggcacgcttgcggcgagtg

SEQ ID NO: 744 - DNA, 20 bp, Bos taurus
cctgccagtatctcaaaccg

SEQ ID NO: 745 - DNA, 23 bp, Homo sapiens
cacatcgatgtcctccccattcc

SEQ ID NO: 746 - DNA, 20 bp, Homo sapiens
atggggaggacatcgatgtc

SEQ ID NO: 747 - RNA, 20 nt, Artificial Sequence
  source: /note="Description of Artificial Sequence: Synthetic oligonucleotide"
cacaucgauguccuccccau

SEQ ID NO: 748 - DNA, 24 bp, Artificial Sequence
  source: /note="Description of Artificial Sequence: Synthetic oligonucleotide"
caccgacatcgatgtcctccccat

SEQ ID NO: 749 - DNA, 24 bp, Artificial Sequence
  source: /note="Description of Artificial Sequence: Synthetic oligonucleotide"
aaacatggggaggacatcgatgtc

SEQ ID NO: 750 - DNA, 26 bp, Artificial Sequence
  source: /note="Description of Artificial Sequence: Synthetic oligonucleotide"
gagggcctatttcccatgattccttc

SEQ ID NO: 751 - DNA, 125 bp, Artificial Sequence
  source: /note="Description of Artificial Sequence: Synthetic polynucleotide"
aaaaaaagcaccgactcggtgccactttttcaagttgataacggactagccttattttaacttgctatttctagctctaaaacatggggaggacatcgatgtcggtgtttcgtcctttccacaag

SEQ ID NO: 752 - DNA, 23 bp, Homo sapiens
cacataggtgtcctccccatagg

SEQ ID NO: 753 - DNA, 23 bp, Homo sapiens
gaaatcaaggtcctccccatagg

SEQ ID NO: 754 - DNA, 23 bp, Homo sapiens
aacttccatctcctccccatggg

SEQ ID NO: 755 - DNA, 23 bp, Homo sapiens
gccttctctgtcctccccatggg

SEQ ID NO: 756 - DNA, 23 bp, Homo sapiens
gagacccatttcctccccattag

SEQ ID NO: 757 - DNA, 23 bp, Homo sapiens
aaaaacaatgtcctccccattag

SEQ ID NO: 758 - DNA, 23 bp, Homo sapiens
gccctcgctgccctccccatcag

SEQ ID NO: 759 - DNA, 23 bp, Homo sapiens
cacggctgtgtcctccccattgg

SEQ ID NO: 760 - DNA, 23 bp, Homo sapiens
tgcttcactgtcctccccatagg

SEQ ID NO: 761 - DNA, 23 bp, Homo sapiens
gtcaacgttgtcctcctcattgg

SEQ ID NO: 762 - DNA, 23 bp, Artificial Sequence
  source: /note="Description of Artificial Sequence: Synthetic primer"
gagggcctatttcccatgattcc

SEQ ID NO: 763 - DNA, 23 bp, Artificial Sequence
  source: /note="Description of Artificial Sequence: Synthetic oligonucleotide"
gagggcctatttcccatgattcc

SEQ ID NO: 764 - DNA, 22 bp, Artificial Sequence
  source: /note="Description of Artificial Sequence: Synthetic oligonucleotide"
cttgtggaaaggacgaaacacc

SEQ ID NO: 765 - DNA, 45 bp, Artificial Sequence
  source: /note="Description of Artificial Sequence: Synthetic oligonucleotide"
  modified_base (4)..(23): a, c, t, g, unknown or other
aacnnnnnnnnnnnnnnnnnnnnggtgtttcgtcctttccacaag

SEQ ID NO: 766 - DNA, 25 bp, Artificial Sequence
  source: /note="Description of Artificial Sequence: Synthetic oligonucleotide"
  modified_base (6)..(25): a, c, t, g, unknown or other
caccgnnnnnnnnnnnnnnnnnnnn

SEQ ID NO: 767 - DNA, 25 bp, Artificial Sequence
  source: /note="Description of Artificial Sequence: Synthetic oligonucleotide"
  modified_base (5)..(24): a, c, t, g, unknown or other
aaacnnnnnnnnnnnnnnnnnnnnc

SEQ ID NO: 768 - DNA, 54 bp, Artificial Sequence
  source: /note="Description of Artificial Sequence: Synthetic oligonucleotide"
aacaccgggtcttcgagaagacctgttttagagctagaaatagcaagttaaaat

SEQ ID NO: 769 - RNA, 20 nt, Artificial Sequence
  source: /note="Description of Artificial Sequence: Synthetic oligonucleotide"
gaguccgagcagaagaagaa

SEQ ID NO: 770 - RNA, 20 nt, Artificial Sequence
  source: /note="Description of Artificial Sequence: Synthetic oligonucleotide"
gucaccuccaaugacuaggg

SEQ ID NO: 771 - RNA, 20 nt, Artificial Sequence
  source: /note="Description of Artificial Sequence: Synthetic oligonucleotide"
gucaccuccaaugacuagaa

SEQ ID NO: 772 - RNA, 20 nt, Artificial Sequence
  source: /note="Description of Artificial Sequence: Synthetic oligonucleotide"
gucaccuccaaugacugagg

SEQ ID NO: 773 - RNA, 20 nt, Artificial Sequence
  source: /note="Description of Artificial Sequence: Synthetic oligonucleotide"
gucaccuccaaugaucaggg

SEQ ID NO: 774 - RNA, 20 nt, Artificial Sequence
  source: /note="Description of Artificial Sequence: Synthetic oligonucleotide"
gucaccuccaauagcuaggg

SEQ ID NO: 775 - RNA, 20 nt, Artificial Sequence
  source: /note="Description of Artificial Sequence: Synthetic oligonucleotide"
gucaccuccagcgacuaggg

SEQ ID NO: 776 - RNA, 20 nt, Artificial Sequence
  source: /note="Description of Artificial Sequence: Synthetic oligonucleotide"
gucaccucugaugacuaggg

SEQ ID NO: 777 - RNA, 20 nt, Artificial Sequence
  source: /note="Description of Artificial Sequence: Synthetic oligonucleotide"
gucacccucaaugacuaggg

SEQ ID NO: 778 - RNA, 20 nt, Artificial Sequence
  source: /note="Description of Artificial Sequence: Synthetic oligonucleotide"
gucauuuccaaugacuaggg

SEQ ID NO: 779 - RNA, 20 nt, Artificial Sequence
  source: /note="Description of Artificial Sequence: Synthetic oligonucleotide"
guugccuccaaugacuaggg

SEQ ID NO: 780 - RNA, 20 nt, Artificial Sequence
  source: /note="Description of Artificial Sequence: Synthetic oligonucleotide"
gucaccuccaaugacugaag

SEQ ID NO: 781 - RNA, 20 nt, Artificial Sequence
  source: /note="Description of Artificial Sequence: Synthetic oligonucleotide"
gucaccuccaauggucaggg

SEQ ID NO: 782 - RNA, 20 nt, Artificial Sequence
  source: /note="Description of Artificial Sequence: Synthetic oligonucleotide"
gucaccuccagcaacuaggg

SEQ ID NO: 783 - RNA, 20 nt, Artificial Sequence
  source: /note="Description of Artificial Sequence: Synthetic oligonucleotide"
gucaccuucgaugacuaggg

SEQ ID NO: 784 - RNA, 20 nt, Artificial Sequence
  source: /note="Description of Artificial Sequence: Synthetic oligonucleotide"
gucauucccaaugacuaggg

SEQ ID NO: 785 - RNA, 20 nt, Artificial Sequence
  source: /note="Description of Artificial Sequence: Synthetic oligonucleotide"
gcugccuccaaugacuaggg

SEQ ID NO: 786 - RNA, 20 nt, Artificial Sequence
  source: /note="Description of Artificial Sequence: Synthetic oligonucleotide"
gucaccuccaaugaccgaaa

SEQ ID NO: 787 - RNA, 20 nt, Artificial Sequence
  source: /note="Description of Artificial Sequence: Synthetic oligonucleotide"
gucaccuccaauagucgggg

SEQ ID NO: 788 - RNA, 20 nt, Artificial Sequence
  source: /note="Description of Artificial Sequence: Synthetic oligonucleotide"
gucaccuccggcagcuaggg

SEQ ID NO: 789 - RNA, 20 nt, Artificial Sequence
  source: /note="Description of Artificial Sequence: Synthetic oligonucleotide"
gucacccuuggugacuaggg

SEQ ID NO: 790 - RNA, 20 nt, Artificial Sequence
  source: /note="Description of Artificial Sequence: Synthetic oligonucleotide"
gucguucucaaugacuaggg

SEQ ID NO: 791 - RNA, 20 nt, Artificial Sequence
  source: /note="Description of Artificial Sequence: Synthetic oligonucleotide"
gacaucgauguccuccccau

SEQ ID NO: 792 - RNA, 20 nt, Artificial Sequence
  source: /note="Description of Artificial Sequence: Synthetic oligonucleotide"
gacaucgauguccuccccgc

SEQ ID NO: 793 - RNA, 20 nt, Artificial Sequence
  source: /note="Description of Artificial Sequence: Synthetic oligonucleotide"
gacaucgauguccuccuuau

SEQ ID NO: 794 - RNA, 20 nt, Artificial Sequence
  source: /note="Description of Artificial Sequence: Synthetic oligonucleotide"
gacaucgauguccuuuccau

SEQ ID NO: 795 - RNA, 20 nt, Artificial Sequence
  source: /note="Description of Artificial Sequence: Synthetic oligonucleotide"
gacaucgaugucucccccau

SEQ ID NO: 796 - RNA, 20 nt, Artificial Sequence
  source: /note="Description of Artificial Sequence: Synthetic oligonucleotide"
gacaucgaugcucuccccau

SEQ ID NO: 797 - RNA, 20 nt, Artificial Sequence
  source: /note="Description of Artificial Sequence: Synthetic oligonucleotide"
gacaucgacauccuccccau

SEQ ID NO: 798 - RNA, 20 nt, Artificial Sequence
  source: /note="Description of Artificial Sequence: Synthetic oligonucleotide"
gacaucaguguccuccccau

SEQ ID NO: 799 - RNA, 20 nt, Artificial Sequence
  source: /note="Description of Artificial Sequence: Synthetic oligonucleotide"
gacacugauguccuccccau

SEQ ID NO: 800 - RNA, 20 nt, Artificial Sequence
  source: /note="Description of Artificial Sequence: Synthetic oligonucleotide"
gaugucgauguccuccccau

SEQ ID NO: 801 - RNA, 20 nt, Artificial Sequence
  source: /note="Description of Artificial Sequence: Synthetic oligonucleotide"
gacaucgauguccuccuugu

SEQ ID NO: 802 - RNA, 20 nt, Artificial Sequence
  source: /note="Description of Artificial Sequence: Synthetic oligonucleotide"
gacaucgaugucccuuccau

SEQ ID NO: 803 - RNA, 20 nt, Artificial Sequence
  source: /note="Description of Artificial Sequence: Synthetic oligonucleotide"
gacaucgaugcuuuccccau

SEQ ID NO: 804 - RNA, 20 nt, Artificial Sequence
  source: /note="Description of Artificial Sequence: Synthetic oligonucleotide"
gacaucggcauccuccccau

SEQ ID NO: 805 - RNA, 20 nt, Artificial Sequence
  source: /note="Description of Artificial Sequence: Synthetic oligonucleotide"
gacacuaauguccuccccau

SEQ ID NO: 806 - RNA, 20 nt, Artificial Sequence
  source: /note="Description of Artificial Sequence: Synthetic oligonucleotide"
ggugucgauguccuccccau

SEQ ID NO: 807 - RNA, 20 nt, Artificial Sequence
  source: /note="Description of Artificial Sequence: Synthetic oligonucleotide"
gacaucgauguccucuuugc

SEQ ID NO: 808 - RNA, 20 nt, Artificial Sequence
  source: /note="Description of Artificial Sequence: Synthetic oligonucleotide"
gacaucgaugucucuuucau

SEQ ID NO: 809 - RNA, 20 nt, Artificial Sequence
  source: /note="Description of Artificial Sequence: Synthetic oligonucleotide"
gacaucgauacuucccccau

SEQ ID NO: 810 - RNA, 20 nt, Artificial Sequence
  source: /note="Description of Artificial Sequence: Synthetic oligonucleotide"
gacaucagcacccuccccau

SEQ ID NO: 811 - RNA, 20 nt, Artificial Sequence
  source: /note="Description of Artificial Sequence: Synthetic oligonucleotide"
gacgcuaguguccuccccau

SEQ ID NO: 812 - RNA, 20 nt, Artificial Sequence
  source: /note="Description of Artificial Sequence: Synthetic oligonucleotide"
gaguccgagcagaagaagaa

SEQ ID NO: 813 - RNA, 20 nt, Artificial Sequence
  source: /note="Description of Artificial Sequence: Synthetic oligonucleotide"
gaguccgagcagaagaaggg

SEQ ID NO: 814 - RNA, 20 nt, Artificial Sequence
  source: /note="Description of Artificial Sequence: Synthetic oligonucleotide"
gaguccgagcagaagagaaa

SEQ ID NO: 815 - RNA, 20 nt, Artificial Sequence
  source: /note="Description of Artificial Sequence: Synthetic oligonucleotide"
gaguccgagcagaaagagaa

SEQ ID NO: 816 - RNA, 20 nt, Artificial Sequence
  source: /note="Description of Artificial Sequence: Synthetic oligonucleotide"
gaguccgagcaggggaagaa

SEQ ID NO: 817 - RNA, 20 nt, Artificial Sequence
  source: /note="Description of Artificial Sequence: Synthetic oligonucleotide"
gaguccgagcgaaagaagaa

SEQ ID NO: 818 - RNA, 20 nt, Artificial Sequence
  source: /note="Description of Artificial Sequence: Synthetic oligonucleotide"
gaguccgaauagaagaagaa

SEQ ID NO: 819 - RNA, 20 nt, Artificial Sequence
  source: /note="Description of Artificial Sequence: Synthetic oligonucleotide"
gaguccaggcagaagaagaa

SEQ ID NO: 820 - RNA, 20 nt, Artificial Sequence
  source: /note="Description of Artificial Sequence: Synthetic oligonucleotide"
gagucugagcagaagaagaa

SEQ ID NO: 821 - RNA, 20 nt, Artificial Sequence
  source: /note="Description of Artificial Sequence: Synthetic oligonucleotide"
gaacccgagcagaagaagaa

SEQ ID NO: 822 - RNA, 20 nt, Artificial Sequence
  source: /note="Description of Artificial Sequence: Synthetic oligonucleotide"
gaguccgagcagaagagaga

SEQ ID NO: 823 - RNA, 20 nt, Artificial Sequence
  source: /note="Description of Artificial Sequence: Synthetic oligonucleotide"
gaguccgagcagagagagaa

SEQ ID NO: 824 - RNA, 20 nt, Artificial Sequence
  source: /note="Description of Artificial Sequence: Synthetic oligonucleotide"
gaguccgagcgagagaagaa

SEQ ID NO: 825 - RNA, 20 nt, Artificial Sequence
  source: /note="Description of Artificial Sequence: Synthetic oligonucleotide"
gaguccggauagaagaagaa

SEQ ID NO: 826 - RNA, 20 nt, Artificial Sequence
  source: /note="Description of Artificial Sequence: Synthetic oligonucleotide"
gagucuaagcagaagaagaa

SEQ ID NO: 827 - RNA, 20 nt, Artificial Sequence
  source: /note="Description of Artificial Sequence: Synthetic oligonucleotide"
ggacccgagcagaagaagaa

SEQ ID NO: 828 - RNA, 20 nt, Artificial Sequence
  source: /note="Description of Artificial Sequence: Synthetic oligonucleotide"
gaguccgagcagaagggagg

SEQ ID NO: 829 - RNA, 20 nt, Artificial Sequence
  source: /note="Description of Artificial Sequence: Synthetic oligonucleotide"
gaguccgagcagggagggaa

SEQ ID NO: 830 - RNA, 20 nt, Artificial Sequence
  source: /note="Description of Artificial Sequence: Synthetic oligonucleotide"
gaguccgagugagggaagaa

SEQ ID NO: 831 - RNA, 20 nt, Artificial Sequence
  source: /note="Description of Artificial Sequence: Synthetic oligonucleotide"
gaguccagauggaagaagaa

SEQ ID NO: 832 - RNA, 20 nt, Artificial Sequence
  source: /note="Description of Artificial Sequence: Synthetic oligonucleotide"
gagccuaggcagaagaagaa

SEQ ID NO: 833 - RNA, 20 nt, Artificial Sequence
  source: /note="Description of Artificial Sequence: Synthetic oligonucleotide"
gcgccaccgguugaugugau

SEQ ID NO: 834 - RNA, 20 nt, Artificial Sequence
  source: /note="Description of Artificial Sequence: Synthetic oligonucleotide"
gcgccaccgguugauguggc

SEQ ID NO: 835 - RNA, 20 nt, Artificial Sequence
  source: /note="Description of Artificial Sequence: Synthetic oligonucleotide"
gcgccaccgguugaugcaau

SEQ ID NO: 836 - RNA, 20 nt, Artificial Sequence
  source: /note="Description of Artificial Sequence: Synthetic oligonucleotide"
gcgccaccgguugacaugau

SEQ ID NO: 837 - RNA, 20 nt, Artificial Sequence
  source: /note="Description of Artificial Sequence: Synthetic oligonucleotide"
gcgccaccgguuagugugau

SEQ ID NO: 838 - RNA, 20 nt, Artificial Sequence
  source: /note="Description of Artificial Sequence: Synthetic oligonucleotide"
gcgccaccggccgaugugau

SEQ ID NO: 839 - RNA, 20 nt, Artificial Sequence
  source: /note="Description of Artificial Sequence: Synthetic oligonucleotide"
gcgccaccaauugaugugau

SEQ ID NO: 840 - RNA, 20 nt, Artificial Sequence
  source: /note="Description of Artificial Sequence: Synthetic oligonucleotide"
gcgccauugguugaugugau

SEQ ID NO: 841 - RNA, 20 nt, Artificial Sequence
  source: /note="Description of Artificial Sequence: Synthetic oligonucleotide"
gcgcugccgguugaugugau

SEQ ID NO: 842 - RNA, 20 nt, Artificial Sequence
  source: /note="Description of Artificial Sequence: Synthetic oligonucleotide"
gcaucaccgguugaugugau

SEQ ID NO: 843 - RNA, 20 nt, Artificial Sequence
  source: /note="Description of Artificial Sequence: Synthetic oligonucleotide"
gcgccaccgguugaugcagu

SEQ ID NO: 844 - RNA, 20 nt, Artificial Sequence
  source: /note="Description of Artificial Sequence: Synthetic oligonucleotide"
gcgccaccgguuggcaugau

SEQ ID NO: 845 - RNA, 20 nt, Artificial Sequence
  source: /note="Description of Artificial Sequence: Synthetic oligonucleotide"
gcgccaccggccaaugugau

SEQ ID NO: 846 - RNA, 20 nt, Artificial Sequence
  source: /note="Description of Artificial Sequence: Synthetic oligonucleotide"
gcgccacuaauugaugugau

SEQ ID NO: 847 - RNA, 20 nt, Artificial Sequence
  source: /note="Description of Artificial Sequence: Synthetic oligonucleotide"
gcgcugucgguugaugugau

SEQ ID NO: 848 - RNA, 20 nt, Artificial Sequence
  source: /note="Description of Artificial Sequence: Synthetic oligonucleotide"
guaucaccgguugaugugau

SEQ ID NO: 849 - RNA, 20 nt, Artificial Sequence
  source: /note="Description of Artificial Sequence: Synthetic oligonucleotide"
gcgccaccgguugauacagc

SEQ ID NO: 850 - RNA, 20 nt, Artificial Sequence
  source: /note="Description of Artificial Sequence: Synthetic oligonucleotide"
gcgccaccgguuagcacgau

SEQ ID NO: 851 - RNA, 20 nt, Artificial Sequence
  source: /note="Description of Artificial Sequence: Synthetic oligonucleotide"
gcgccaccgaccagugugau

SEQ ID NO: 852 - RNA, 20 nt, Artificial Sequence
  source: /note="Description of Artificial Sequence: Synthetic oligonucleotide"
gcgccauuaacugaugugau

SEQ ID NO: 853 - RNA, 20 nt, Artificial Sequence
  source: /note="Description of Artificial Sequence: Synthetic oligonucleotide"
gcguuguugguugaugugau

SEQ ID NO: 854 - RNA, 20 nt, Artificial Sequence
  source: /note="Description of Artificial Sequence: Synthetic oligonucleotide"
gucaccuccaaugacuaggg

SEQ ID NO: 855 - RNA, 20 nt, Artificial Sequence
  source: /note="Description of Artificial Sequence: Synthetic oligonucleotide"
gucaccuccaaugacuaaga

SEQ ID NO: 856 - RNA, 20 nt, Artificial Sequence
  source: /note="Description of Artificial Sequence: Synthetic oligonucleotide"
gucaccuccaaugauuagga

SEQ ID NO: 857 - RNA, 20 nt, Artificial Sequence
  source: /note="Description of Artificial Sequence: Synthetic oligonucleotide"
gucaccuccagugacuagga

SEQ ID NO: 858 - RNA, 20 nt, Artificial Sequence
  source: /note="Description of Artificial Sequence: Synthetic oligonucleotide"
gucacuuccaaugacuagga

SEQ ID NO: 859 - RNA, 20 nt, Artificial Sequence
  source: /note="Description of Artificial Sequence: Synthetic oligonucleotide"
aucaccuccaaugacuagga

SEQ ID NO: 860 - RNA, 20 nt, Artificial Sequence
  source: /note="Description of Artificial Sequence: Synthetic oligonucleotide"
gucaccuccaaugaccaagg

SEQ ID NO: 861 - RNA, 20 nt, Artificial Sequence
  source: /note="Description of Artificial Sequence: Synthetic oligonucleotide"
gucaccuccaauaacuaagg

SEQ ID NO: 862 - RNA, 20 nt, Artificial Sequence
  source: /note="Description of Artificial Sequence: Synthetic oligonucleotide"
gucaccucuaaugacuaagg

SEQ ID NO: 863 - RNA, 20 nt, Artificial Sequence
  source: /note="Description of Artificial Sequence: Synthetic oligonucleotide"
gucgccuccaaugacuaagg

SEQ ID NO: 864 - RNA, 20 nt, Artificial Sequence
  source: /note="Description of Artificial Sequence: Synthetic oligonucleotide"
gucaccuccaauggccaggg

SEQ ID NO: 865 - RNA, 20 nt, Artificial Sequence
  source: /note="Description of Artificial Sequence: Synthetic oligonucleotide"
gucaccuccagugaccaggg

SEQ ID NO: 866 - RNA, 20 nt, Artificial Sequence
  source: /note="Description of Artificial Sequence: Synthetic oligonucleotide"
gucacccccaaugaccaggg

SEQ ID NO: 867 - RNA, 20 nt, Artificial Sequence
  source: /note="Description of Artificial Sequence: Synthetic oligonucleotide"
gccaccuccaaugaccaggg

SEQ ID NO: 868 - RNA, 20 nt, Artificial Sequence
  source: /note="Description of Artificial Sequence: Synthetic oligonucleotide"
gacaucgauguccuccccau

SEQ ID NO: 869 - RNA, 20 nt, Artificial Sequence
  source: /note="Description of Artificial Sequence: Synthetic oligonucleotide"
gacaucgauguccucccuag

SEQ ID NO: 870 - RNA, 20 nt, Artificial Sequence
  source: /note="Description of Artificial Sequence: Synthetic oligonucleotide"
gacaucgauguccuucccag

SEQ ID NO: 871 - RNA, 20 nt, Artificial Sequence
  source: /note="Description of Artificial Sequence: Synthetic oligonucleotide"
gacaucgaugcccuccccag

SEQ ID NO: 872 - RNA, 20 nt, Artificial Sequence
  source: /note="Description of Artificial Sequence: Synthetic oligonucleotide"
gacauugauguccuccccag

SEQ ID NO: 873 - RNA, 20 nt, Artificial Sequence
  source: /note="Description of Artificial Sequence: Synthetic oligonucleotide"
aacaucgauguccuccccag

SEQ ID NO: 874 - RNA, 20 nt, Artificial Sequence
  source: /note="Description of Artificial Sequence: Synthetic oligonucleotide"
gacaucgauguccucucuau

SEQ ID NO: 875 - RNA, 20 nt, Artificial Sequence
  source: /note="Description of Artificial Sequence: Synthetic oligonucleotide"
gacaucgaugucuucccuau

SEQ ID NO: 876 - RNA, 20 nt, Artificial Sequence
  source: /note="Description of Artificial Sequence: Synthetic oligonucleotide"
gacaucgacguccucccuau

SEQ ID NO: 877 - RNA, 20 nt, Artificial Sequence
  source: /note="Description of Artificial Sequence: Synthetic oligonucleotide"
gacgucgauguccucccuau

SEQ ID NO: 878 - RNA, 20 nt, Artificial Sequence
  source: /note="Description of Artificial Sequence: Synthetic oligonucleotide"
gacaucgauguccccuccau

SEQ ID NO: 879 - RNA, 20 nt, Artificial Sequence
  source: /note="Description of Artificial Sequence: Synthetic oligonucleotide"
gacaucgaugcccucuccau

SEQ ID NO: 880 - RNA, 20 nt, Artificial Sequence
  source: /note="Description of Artificial Sequence: Synthetic oligonucleotide"
gacaucaauguccucuccau

SEQ ID NO: 881 - RNA, 20 nt, Artificial Sequence
  source: /note="Description of Artificial Sequence: Synthetic oligonucleotide"
ggcaucgauguccucuccau

SEQ ID NO: 882 - RNA, 20 nt, Artificial Sequence
  source: /note="Description of Artificial Sequence: Synthetic oligonucleotide"
gaguccgagcagaagaagaa

SEQ ID NO: 883 - RNA, 20 nt, Artificial Sequence
  source: /note="Description of Artificial Sequence: Synthetic oligonucleotide"
gaguccgagcagaagaaaag

SEQ ID NO: 884 - RNA, 20 nt, Artificial Sequence
  source: /note="Description of Artificial Sequence: Synthetic oligonucleotide"
gaguccgagcagaaaaagag

SEQ ID NO: 885 - RNA, 20 nt, Artificial Sequence
  source: /note="Description of Artificial Sequence: Synthetic oligonucleotide"
gaguccgagcggaagaagag

SEQ ID NO: 886 - RNA, 20 nt, Artificial Sequence
  source: /note="Description of Artificial Sequence: Synthetic oligonucleotide"
gagucugagcagaagaagag

SEQ ID NO: 887 - RNA, 20 nt, Artificial Sequence
  source: /note="Description of Artificial Sequence: Synthetic oligonucleotide"
aaguccgagcagaagaagag

SEQ ID NO: 888 - RNA, 20 nt, Artificial Sequence
  source: /note="Description of Artificial Sequence: Synthetic oligonucleotide"
gaguccgagcagaagcaaaa

SEQ ID NO: 889 - RNA, 20 nt, Artificial Sequence
  source: /note="Description of Artificial Sequence: Synthetic oligonucleotide"
gaguccgagcaggagaaaaa

SEQ ID NO: 890 - RNA, 20 nt, Artificial Sequence
  source: /note="Description of Artificial Sequence: Synthetic oligonucleotide"
gaguccgaacagaagaaaaa

SEQ ID NO: 891 - RNA, 20 nt, Artificial Sequence
  source: /note="Description of Artificial Sequence: Synthetic oligonucleotide"
gagcccgagcagaagaaaaa

SEQ ID NO: 892 - RNA, 20 nt, Artificial Sequence
  source: /note="Description of Artificial Sequence: Synthetic oligonucleotide"
gaguccgagcagagggagaa

SEQ ID NO: 893 - RNA, 20 nt, Artificial Sequence
  source: /note="Description of Artificial Sequence: Synthetic oligonucleotide"
gaguccgagcggaaggagaa

SEQ ID NO: 894 - RNA, 20 nt, Artificial Sequence
  source: /note="Description of Artificial Sequence: Synthetic oligonucleotide"
gaguccaagcagaaggagaa

SEQ ID NO: 895 - RNA, 20 nt, Artificial Sequence
  source: /note="Description of Artificial Sequence: Synthetic oligonucleotide"
ggguccgagcagaaggagaa

SEQ ID NO: 896 - RNA, 20 nt, Artificial Sequence
  source: /note="Description of Artificial Sequence: Synthetic oligonucleotide"
gcgccaccgguugaugugau

SEQ ID NO: 897 - RNA, 20 nt, Artificial Sequence
  source: /note="Description of Artificial Sequence: Synthetic oligonucleotide"
gcgccaccgguugauguaac

SEQ ID NO: 898 - RNA, 20 nt, Artificial Sequence
  source: /note="Description of Artificial Sequence: Synthetic oligonucleotide"
gcgccaccgguugaugugac

SEQ ID NO: 899 - RNA, 20 nt, Artificial Sequence
  source: /note="Description of Artificial Sequence: Synthetic oligonucleotide"
gcgccaccggcugaugugac

SEQ ID NO: 900 - RNA, 20 nt, Artificial Sequence
  source: /note="Description of Artificial Sequence: Synthetic oligonucleotide"
gcgccgccgguugaugugac

SEQ ID NO: 901 - RNA, 20 nt, Artificial Sequence
  source: /note="Description of Artificial Sequence: Synthetic oligonucleotide"
acgccaccgguugaugugac

SEQ ID NO: 902 - RNA, 20 nt, Artificial Sequence
  source: /note="Description of Artificial Sequence: Synthetic oligonucleotide"
gcgccaccgguugauauaau

SEQ ID NO: 903 - RNA, 20 nt, Artificial Sequence
  source: /note="Description of Artificial Sequence: Synthetic oligonucleotide"
gcgccaccgguuaauguaau

SEQ ID NO: 904 - RNA, 20 nt, Artificial Sequence
  source: /note="Description of Artificial Sequence: Synthetic oligonucleotide"
gcgccaccaguugauguaau

SEQ ID NO: 905 - RNA, 20 nt, Artificial Sequence
  source: /note="Description of Artificial Sequence: Synthetic oligonucleotide"
gcgucaccgguugauguaau

SEQ ID NO: 906 - RNA, 20 nt, Artificial Sequence
  source: /note="Description of Artificial Sequence: Synthetic oligonucleotide"
gcgccaccgguugguaugau

SEQ ID NO: 907 - RNA, 20 nt, Artificial Sequence
  source: /note="Description of Artificial Sequence: Synthetic oligonucleotide"
gcgccaccggcugauaugau

SEQ ID NO: 908 - RNA, 20 nt, Artificial Sequence
  source: /note="Description of Artificial Sequence: Synthetic oligonucleotide"
gcgccaucgguugauaugau

SEQ ID NO: 909 - RNA, 20 nt, Artificial Sequence
  source: /note="Description of Artificial Sequence: Synthetic oligonucleotide"
gugccaccgguugauaugau

SEQ ID NO: 910 - RNA, 20 nt, Artificial Sequence
  source: /note="Description of Artificial Sequence: Synthetic oligonucleotide"
gucaccuccaaugacuaggg

SEQ ID NO: 911 - RNA, 20 nt, Artificial Sequence
  source: /note="Description of Artificial Sequence: Synthetic oligonucleotide"
gucaccuccaaugaccaaga

SEQ ID NO: 912 - RNA, 20 nt, Artificial Sequence
  source: /note="Description of Artificial Sequence: Synthetic oligonucleotide"
gucaccuccaauggcuggga

SEQ ID NO: 913 - RNA, 20 nt, Artificial Sequence
  source: /note="Description of Artificial Sequence: Synthetic oligonucleotide"
gucaccuccaacgaccagga

SEQ ID NO: 914 - RNA, 20 nt, Artificial Sequence
  source: /note="Description of Artificial Sequence: Synthetic oligonucleotide"
gucaccuccgaugauuagga

SEQ ID NO: 915 - RNA, 20 nt, Artificial Sequence
  source: /note="Description of Artificial Sequence: Synthetic oligonucleotide"
gucaccuccaauggccaagg

SEQ ID NO: 916 - RNA, 20 nt, Artificial Sequence
  source: /note="Description of Artificial Sequence: Synthetic oligonucleotide"
gucaccuccaacgauuaagg

SEQ ID NO: 917 - RNA, 20 nt, Artificial Sequence
  source: /note="Description of Artificial Sequence: Synthetic oligonucleotide"
gucaccuccgauggcuaagg

SEQ ID NO: 918 - RNA, 20 nt, Artificial Sequence
  source: /note="Description of Artificial Sequence: Synthetic oligonucleotide"
gucaccuucaauaacuaagg

SEQ ID NO: 919 - RNA, 20 nt, Artificial Sequence
  source: /note="Description of Artificial Sequence: Synthetic oligonucleotide"
gucaccuccaauggccaaga

SEQ ID NO: 920 - RNA, 20 nt, Artificial Sequence
  source: /note="Description of Artificial Sequence: Synthetic oligonucleotide"
gucaccuccaguggcuggga

SEQ ID NO: 921 - RNA, 20 nt, Artificial Sequence
  source: /note="Description of Artificial Sequence: Synthetic oligonucleotide"
gucaccuucaacgaccagga

SEQ ID NO: 922 - RNA, 20 nt, Artificial Sequence
  source: /note="Description of Artificial Sequence: Synthetic oligonucleotide"
gucaucuccgaugauuagga

SEQ ID NO: 923 - RNA, 20 nt, Artificial Sequence
  source: /note="Description of Artificial Sequence: Synthetic oligonucleotide"
gccaccuucaauggcuagga

SEQ ID NO: 924 - RNA, 20 nt, Artificial Sequence
  source: /note="Description of Artificial Sequence: Synthetic oligonucleotide"
gacaucgauguccuccccau

SEQ ID NO: 925 - RNA, 20 nt, Artificial Sequence
  source: /note="Description of Artificial Sequence: Synthetic oligonucleotide"
gacaucgauguccucucuag

SEQ ID NO: 926 - RNA, 20 nt, Artificial Sequence
  source: /note="Description of Artificial Sequence: Synthetic oligonucleotide"
gacaucgaugucccccucag

SEQ ID NO: 927 - RNA, 20 nt, Artificial Sequence
  source: /note="Description of Artificial Sequence: Synthetic oligonucleotide"
gacaucgauguucucuccag

SEQ ID NO: 928 - RNA, 20 nt, Artificial Sequence
  source: /note="Description of Artificial Sequence: Synthetic oligonucleotide"
gacaucgauauccuucccag

SEQ ID NO: 929 - RNA, 20 nt, Artificial Sequence
  source: /note="Description of Artificial Sequence: Synthetic oligonucleotide"
gacaucgauguccccucuau

SEQ ID NO: 930 - RNA, 20 nt, Artificial Sequence
  source: /note="Description of Artificial Sequence: Synthetic oligonucleotide"
gacaucgauguucuuccuau

SEQ ID NO: 931 - RNA, 20 nt, Artificial Sequence
  source: /note="Description of Artificial Sequence: Synthetic oligonucleotide"
gacaucgauauccccccuau

SEQ ID NO: 932 - RNA, 20 nt, Artificial Sequence
  source: /note="Description of Artificial Sequence: Synthetic oligonucleotide"
gacaucggugucaucccuau

SEQ ID NO: 933 - RNA, 20 nt, Artificial Sequence
  source: /note="Description of Artificial Sequence: Synthetic oligonucleotide"
gacaucgauguccccucuag

SEQ ID NO: 934 - RNA, 20 nt, Artificial Sequence
  source: /note="Description of Artificial Sequence: Synthetic oligonucleotide"
gacaucgaugccccccucag

SEQ ID NO: 935 - RNA, 20 nt, Artificial Sequence
  source: /note="Description of Artificial Sequence: Synthetic oligonucleotide"
gacaucgguguucucuccag

SEQ ID NO: 936 - RNA, 20 nt, Artificial Sequence
  source: /note="Description of Artificial Sequence: Synthetic oligonucleotide"
gacaccgauauccuucccag

SEQ ID NO: 937 - RNA, 20 nt, Artificial Sequence
  source: /note="Description of Artificial Sequence: Synthetic oligonucleotide"
ggcaucggugucccccccag

SEQ ID NO: 938 - RNA, 20 nt, Artificial Sequence
  source: /note="Description of Artificial Sequence: Synthetic oligonucleotide"
gaguccgagcagaagaagaa

SEQ ID NO: 939 - RNA, 20 nt, Artificial Sequence
  source: /note="Description of Artificial Sequence: Synthetic oligonucleotide"
gaguccgagcagaaggaaag

SEQ ID NO: 940 - RNA, 20 nt, Artificial Sequence
  source: /note="Description of Artificial Sequence: Synthetic oligonucleotide"
gaguccgagcagaggaggag

SEQ ID NO: 941 - RNA, 20 nt, Artificial Sequence
  source: /note="Description of Artificial Sequence: Synthetic oligonucleotide"
gaguccgagcaaaaggagag

SEQ ID NO: 942 - RNA, 20 nt, Artificial Sequence
  source: /note="Description of Artificial Sequence: Synthetic oligonucleotide"
gaguccgaguagaaaaagag

SEQ ID NO: 943 - RNA, 20 nt, Artificial Sequence
  source: /note="Description of Artificial Sequence: Synthetic oligonucleotide"
gaguccgagcagagggaaaa

SEQ ID NO: 944 - RNA, 20 nt, Artificial Sequence
  source: /note="Description of Artificial Sequence: Synthetic oligonucleotide"
gaguccgagcaaaaaaaaaa

SEQ ID NO: 945 - RNA, 20 nt, Artificial Sequence
  source: /note="Description of Artificial Sequence: Synthetic oligonucleotide"
gaguccgaguagaggaaaaa

SEQ ID NO: 946 - RNA, 20 nt, Artificial Sequence
  source: /note="Description of Artificial Sequence: Synthetic oligonucleotide"
gaguccgggcaggagaaaaa

SEQ ID NO: 947 - RNA, 20 nt, Artificial Sequence
  source: /note="Description of Artificial Sequence: Synthetic oligonucleotide"
gaguccgagcagagggaaag

SEQ ID NO: 948 - RNA, 20 nt, Artificial Sequence
  source: /note="Description of Artificial Sequence: Synthetic oligonucleotide"
gaguccgagcggaggaggag

SEQ ID NO: 949 - RNA, 20 nt, Artificial Sequence
  source: /note="Description of Artificial Sequence: Synthetic oligonucleotide"
gaguccgggcaaaaggagag

SEQ ID NO: 950 - RNA, 20 nt, Artificial Sequence
  source: /note="Description of Artificial Sequence: Synthetic oligonucleotide"
gaguucgaguagaaaaagag

SEQ ID NO: 951 - RNA, 20 nt, Artificial Sequence
  source: /note="Description of Artificial Sequence: Synthetic oligonucleotide"
ggguccgggcagaggaagag

SEQ ID NO: 952 - RNA, 20 nt, Artificial Sequence
  source: /note="Description of Artificial Sequence: Synthetic oligonucleotide"
gcgccaccgguugaugugau

SEQ ID NO: 953 - RNA, 20 nt, Artificial Sequence
  source: /note="Description of Artificial Sequence: Synthetic oligonucleotide"
gcgccaccgguugauauaac

SEQ ID NO: 954 - RNA, 20 nt, Artificial Sequence
  source: /note="Description of Artificial Sequence: Synthetic oligonucleotide"
gcgccaccgguuggugcgac

SEQ ID NO: 955 - RNA, 20 nt, Artificial Sequence
  source: /note="Description of Artificial Sequence: Synthetic oligonucleotide"
gcgccaccggucgauaugac

SEQ ID NO: 956 - RNA, 20 nt, Artificial Sequence
  source: /note="Description of Artificial Sequence: Synthetic oligonucleotide"
gcgccaccgauugacgugac

SEQ ID NO: 957 - RNA, 20 nt, Artificial Sequence
  source: /note="Description of Artificial Sequence: Synthetic oligonucleotide"
gcgccaccgguugguauaau

SEQ ID NO: 958 - RNA, 20 nt, Artificial Sequence
  source: /note="Description of Artificial Sequence: Synthetic oligonucleotide"
gcgccaccggucgacguaau

SEQ ID NO: 959 - RNA, 20 nt, Artificial Sequence
  source: /note="Description of Artificial Sequence: Synthetic oligonucleotide"
gcgccaccgauugguguaau

SEQ ID NO: 960 - RNA, 20 nt, Artificial Sequence
  source: /note="Description of Artificial Sequence: Synthetic oligonucleotide"
gcgccacugguuaauguaau

SEQ ID NO: 961 - RNA, 20 nt, Artificial Sequence
  source: /note="Description of Artificial Sequence: Synthetic oligonucleotide"
gcgccaccgguugguauaac

SEQ ID NO: 962 - RNA, 20 nt, Artificial Sequence
  source: /note="Description of Artificial Sequence: Synthetic oligonucleotide"
gcgccaccggcuggugcgac

SEQ ID NO: 963 - RNA, 20 nt, Artificial Sequence
  source: /note="Description of Artificial Sequence: Synthetic oligonucleotide"
gcgccacuggucgauaugac

SEQ ID NO: 964 - RNA, 20 nt, Artificial Sequence
  source: /note="Description of Artificial Sequence: Synthetic oligonucleotide"
gcgcuaccgauugacgugac

SEQ ID NO: 965 - RNA, 20 nt, Artificial Sequence
  source: /note="Description of Artificial Sequence: Synthetic oligonucleotide"
gugccacugguuggugugac

SEQ ID NO: 966 - RNA, 20 nt, Artificial Sequence
  source: /note="Description of Artificial Sequence: Synthetic oligonucleotide"
gucaccuccaaugacuaggg

SEQ ID NO: 967 - DNA, 23 bp, Artificial Sequence
  source: /note="Description of Artificial Sequence: Synthetic oligonucleotide"
  source: /note="Description of Combined DNA/RNA Molecule: Synthetic oligonucleotide"
gucaccuccaaugacuagggtgg

SEQ ID NO: 968 - DNA, 23 bp, Artificial Sequence
  source: /note="Description of Artificial Sequence: Synthetic oligonucleotide"
  source: /note="Description of Combined DNA/RNA Molecule: Synthetic oligonucleotide"
gucaacuccaaugatuaggacag

SEQ ID NO: 969 - DNA, 23 bp, Artificial Sequence
  source: /note="Description of Artificial Sequence: Synthetic oligonucleotide"
  source: /note="Description of Combined DNA/RNA Molecule: Synthetic oligonucleotide"
gucaccuccacutccuagggcag

SEQ ID NO: 970 - DNA, 23 bp, Artificial Sequence
  source: /note="Description of Artificial Sequence: Synthetic oligonucleotide"
  source: /note="Description of Combined DNA/RNA Molecule: Synthetic oligonucleotide"
gucactuccaaggacuagagaag

SEQ ID NO: 971 - DNA, 23 bp, Artificial Sequence
  source: /note="Description of Artificial Sequence: Synthetic oligonucleotide"
  source: /note="Description of Combined DNA/RNA Molecule: Synthetic oligonucleotide"
gucaccuccagggtcuagggcag

SEQ ID NO: 972 - DNA, 23 bp, Artificial Sequence
  source: /note="Description of Artificial Sequence: Synthetic oligonucleotide"
  source: /note="Description of Combined DNA/RNA Molecule: Synthetic oligonucleotide"
gucaacuccaaugacutgggagg

SEQ ID NO: 973 - DNA, 23 bp, Artificial Sequence
  source: /note="Description of Artificial Sequence: Synthetic oligonucleotide"
  source: /note="Description of Combined DNA/RNA Molecule: Synthetic oligonucleotide"
gucaccutaaaugacutgggaag

SEQ ID NO: 974 - DNA, 23 bp, Artificial Sequence
  source: /note="Description of Artificial Sequence: Synthetic oligonucleotide"
  source: /note="Description of Combined DNA/RNA Molecule: Synthetic oligonucleotide"
tucaccuccaaaaacuagggaag

SEQ ID NO: 975 - DNA, 23 bp, Artificial Sequence
  source: /note="Description of Artificial Sequence: Synthetic oligonucleotide"
  source: /note="Description of Combined DNA/RNA Molecule: Synthetic oligonucleotide"
gctaccuccagugacuagggaag

SEQ ID NO: 976 - DNA, 12 bp, Homo sapiens
tgactagggtgg

SEQ ID NO: 977 - DNA, 11 bp, Homo sapiens
tgactgggtgg

SEQ ID NO: 978 - DNA, 14 bp, Homo sapiens
tgactatagggtgg

SEQ ID NO: 979 - DNA, 12 bp, Homo sapiens
tgactagggaag

SEQ ID NO: 980 - DNA, 11 bp, Homo sapiens
tgactgggaag

SEQ ID NO: 981 - DNA, 14 bp, Homo sapiens
tgactatagggaag

SEQ ID NO: 982 - DNA, 14 bp, Homo sapiens
tgactggagggaag

SEQ ID NO: 983 - DNA, 13 bp, Homo sapiens
tgactacgggaag

SEQ ID NO: 984 - RNA, 20 nt, Artificial Sequence
  source: /note="Description of Artificial Sequence: Synthetic oligonucleotide"
gaguccgagcagaagaagaa

SEQ ID NO: 985 - RNA, 23 nt, Artificial Sequence
  source: /note="Description of Artificial Sequence: Synthetic oligonucleotide"
gaguccgagcagaagaagaaggg

SEQ ID NO: 986 - RNA, 23 nt, Artificial Sequence
  source: /note="Description of Artificial Sequence: Synthetic oligonucleotide"
gaggccgagcagaagaaagacgg

SEQ ID NO: 987 - RNA, 23 nt, Artificial Sequence
  source: /note="Description of Artificial Sequence: Synthetic oligonucleotide"
gagucccagcagaggaagcagag

SEQ ID NO: 988 - DNA, 23 bp, Artificial Sequence
  source: /note="Description of Artificial Sequence: Synthetic oligonucleotide"
  source: /note="Description of Combined DNA/RNA Molecule: Synthetic oligonucleotide"
gaguccaagcagaggaaggatag

SEQ ID NO: 989 - DNA, 23 bp, Artificial Sequence
  source: /note="Description of Artificial Sequence: Synthetic oligonucleotide"
  source: /note="Description of Combined DNA/RNA Molecule: Synthetic oligonucleotide"
gagucagagcagaactagaaggg

SEQ ID NO: 990 - RNA, 23 nt, Artificial Sequence
  source: /note="Description of Artificial Sequence: Synthetic oligonucleotide"
gagucccaggagaagaagagagg

SEQ ID NO: 991 - DNA, 23 bp, Artificial Sequence
  source: /note="Description of Artificial Sequence: Synthetic oligonucleotide"
  source: /note="Description of Combined DNA/RNA Molecule: Synthetic oligonucleotide"
gaguccaagcagtagaggaaggg

SEQ ID NO: 992 - DNA, 23 bp, Artificial Sequence
  source: /note="Description of Artificial Sequence: Synthetic oligonucleotide"
  source: /note="Description of Combined DNA/RNA Molecule: Synthetic oligonucleotide"
gaguccgagaaaatgaagaagag

SEQ ID NO: 993 - RNA, 23 nt, Artificial Sequence
  source: /note="Description of Artificial Sequence: Synthetic oligonucleotide"
gagucccagaagaagaaaaaaag

SEQ ID NO: 994 - RNA, 23 nt, Artificial Sequence
  source: /note="Description of Artificial Sequence: Synthetic oligonucleotide"
gagucccaggagaagaaaaacag

SEQ ID NO: 995 - RNA, 23 nt, Artificial Sequence
  source: /note="Description of Artificial Sequence: Synthetic oligonucleotide"
gagucagaacagaagaacaacag

SEQ ID NO: 996 - DNA, 23 bp, Artificial Sequence
  source: /note="Description of Artificial Sequence: Synthetic oligonucleotide"
  source: /note="Description of Combined DNA/RNA Molecule: Synthetic oligonucleotide"
gaguccaagaagaataagaatag

SEQ ID NO: 997 - RNA, 23 nt, Artificial Sequence
  source: /note="Description of Artificial Sequence: Synthetic oligonucleotide"
gaauccaagcagaagaagagaag

SEQ ID NO: 998 - RNA, 23 nt, Artificial Sequence
  source: /note="Description of Artificial Sequence: Synthetic oligonucleotide"
gagucagaccaggagaagaagag

SEQ ID NO: 999 - RNA, 23 nt, Artificial Sequence
  source: /note="Description of Artificial Sequence: Synthetic oligonucleotide"
aaguccgagaagaagcagaaaag

SEQ ID NO: 1000 - DNA, 23 bp, Artificial Sequence
  source: /note="Description of Artificial Sequence: Synthetic oligonucleotide"
  source: /note="Description of Combined DNA/RNA Molecule: Synthetic oligonucleotide"
gaguctgggcaggagaagaagag

SEQ ID NO: 1001 - DNA, 23 bp, Artificial Sequence
  source: /note="Description of Artificial Sequence: Synthetic oligonucleotide"
  source: /note="Description of Combined DNA/RNA Molecule: Synthetic oligonucleotide"
gaguctgaacggaagaagaaaag

SEQ ID NO: 1002 - DNA, 23 bp, Artificial Sequence
  source: /note="Description of Artificial Sequence: Synthetic oligonucleotide"
  source: /note="Description of Combined DNA/RNA Molecule: Synthetic oligonucleotide"
aaguctgagcagaagaagcacag

SEQ ID NO: 1003 - RNA, 23 nt, Artificial Sequence
  source: /note="Description of Artificial Sequence: Synthetic oligonucleotide"
aaguccgaggagaggaagaaagg

SEQ ID NO: 1004 - RNA, 23 nt, Artificial Sequence
  source: /note="Description of Artificial Sequence: Synthetic oligonucleotide"
gaggcccagcagaggaagaagag

SEQ ID NO: 1005 - DNA, 23 bp, Artificial Sequence
  source: /note="Description of Artificial Sequence: Synthetic oligonucleotide"
  source: /note="Description of Combined DNA/RNA Molecule: Synthetic oligonucleotide"
gagutccagaagaagaagaagag

SEQ ID NO: 1006 - DNA, 23 bp, Artificial Sequence
  source: /note="Description of Artificial Sequence: Synthetic oligonucleotide"
  source: /note="Description of Combined DNA/RNA Molecule: Synthetic oligonucleotide"
gaguactagaagaagaagaaaag

SEQ ID NO: 1007 - DNA, 23 bp, Artificial Sequence
  source: /note="Description of Artificial Sequence: Synthetic oligonucleotide"
  source: /note="Description of Combined DNA/RNA Molecule: Synthetic oligonucleotide"
gacucctagcaaaagaagaatgg

SEQ ID NO: 1008 - DNA, 23 bp, Artificial Sequence
  source: /note="Description of Artificial Sequence: Synthetic oligonucleotide"
  source: /note="Description of Combined DNA/RNA Molecule: Synthetic oligonucleotide"
gaguttgagtagaagaagaagag

SEQ ID NO: 1009 - RNA, 23 nt, Artificial Sequence
  source: /note="Description of Artificial Sequence: Synthetic oligonucleotide"
gaguaagagaagaagaagaaggg

SEQ ID NO: 1010 - RNA, 23 nt, Artificial Sequence
  source: /note="Description of Artificial Sequence: Synthetic oligonucleotide"
gaguaggaggagaagaagaaagg

SEQ ID NO: 1011 - DNA, 23 bp, Artificial Sequence
  source: /note="Description of Artificial Sequence: Synthetic oligonucleotide"
  source: /note="Description of Combined DNA/RNA Molecule: Synthetic oligonucleotide"
gagucctagcaggagaagaagag

SEQ ID NO: 1012 - DNA, 23 bp, Artificial Sequence
  source: /note="Description of Artificial Sequence: Synthetic oligonucleotide"
  source: /note="Description of Combined DNA/RNA Molecule: Synthetic oligonucleotide"
gatucctaccagaagaagaatgg

SEQ ID NO: 1013 - RNA, 23 nt, Artificial Sequence
  source: /note="Description of Artificial Sequence: Synthetic oligonucleotide"
gagucccagcaaaagaagaaaag

SEQ ID NO: 1014 - RNA, 23 nt, Artificial Sequence
  source: /note="Description of Artificial Sequence: Synthetic oligonucleotide"
gagagcaagcagaagaagaaggg

SEQ ID NO: 1015 - RNA, 23 nt, Artificial Sequence
  source: /note="Description of Artificial Sequence: Synthetic oligonucleotide"
aagucagaggagaagaagaaaag

SEQ ID NO: 1016 - DNA, 23 bp, Artificial Sequence
  source: /note="Description of Artificial Sequence: Synthetic oligonucleotide"
  source: /note="Description of Combined DNA/RNA Molecule: Synthetic oligonucleotide"
gaguctaagcagaagaagaagag

SEQ ID NO: 1017 - DNA, 23 bp, Artificial Sequence
  source: /note="Description of Artificial Sequence: Synthetic oligonucleotide"
  source: /note="Description of Combined DNA/RNA Molecule: Synthetic oligonucleotide"
acguctgagcagaagaagaatgg

SEQ ID NO: 1018 - DNA, 12 bp, Homo sapiens
gaagaagaaggg

SEQ ID NO: 1019 - DNA, 13 bp, Homo sapiens
gaagaaggaaggg

SEQ ID NO: 1020 - DNA, 13 bp, Homo sapiens
gaagaaagaaggg

SEQ ID NO: 1021 - DNA, 15 bp, Homo sapiens
gaagaattagaaggg

SEQ ID NO: 1022 - DNA, 14 bp, Homo sapiens
gaagaacagaaggg

SEQ ID NO: 1023 - DNA, 11 bp, Homo sapiens
gaagagaaggg

SEQ ID NO: 1024 - DNA, 11 bp, Homo sapiens
gaagaaaaggg

SEQ ID NO: 1025 - DNA, 12 bp, Homo sapiens
gaagaaagacgg

SEQ ID NO: 1026 - DNA, 11 bp, Homo sapiens
gaagaagacgg

SEQ ID NO: 1027 - DNA, 13 bp, Homo sapiens
gaagaaaagacgg

SEQ ID NO: 1028 - DNA, 13 bp, Homo sapiens
gaagaatagacgg

SEQ ID NO: 1029 - DNA, 13 bp, Homo sapiens
gaagaacagacgg

SEQ ID NO: 1030 - DNA, 14 bp, Homo sapiens
gaagaataagacgg

SEQ ID NO: 1031 - DNA, 12 bp, Homo sapiens
ggagaagaagag

SEQ ID NO: 1032 - DNA, 13 bp, Homo sapiens
ggagaaagaagag

SEQ ID NO: 1033 - DNA, 11 bp, Homo sapiens
ggagagaagag

SEQ ID NO: 1034 - DNA, 11 bp, Homo sapiens
ggagaaaagag

SEQ ID NO: 1035 - DNA, 14 bp, Homo sapiens
ggagaatagaagag

SEQ ID NO: 1036 - DNA, 12 bp, Homo sapiens
gaagaagaagag

SEQ ID NO: 1037 - DNA, 13 bp, Homo sapiens
gaagaaagaagag

SEQ ID NO: 1038 - DNA, 11 bp, Homo sapiens
gaagagaagag

SEQ ID NO: 1039 - DNA, 11 bp, Homo sapiens
gaagaaaagag

SEQ ID NO: 1040 - DNA, 384 bp, Homo sapiens
cccagtggctgctctgggggcctcctgagtttctcatctgtgcccctccctccctggcccaggtgaaggtgtggttccagaaccggaggacaaagtacaaacggcagaagctggaggaggaagggcctgagtccgagcagaagaagaagggctcccatcacatcaaccggtggcgcattgccacgaagcaggccaatggggaggacatcgatgtcacctccaatgactagggtgggcaaccacaaacccacgagggggcagagtgctgcttgctgctggccaggcccctgcgtgggcccaagctggactctggccactccctggccaggctttggggaggcctggagtcatggccccacagggcttgaagcccggggccgccat

SEQ ID NO: 1041 - DNA, 23 bp, Homo sapiens
gtcacctccaatgactagggtgg

SEQ ID NO: 1042 - DNA, 23 bp, Homo sapiens
gacatcgatgtcctccccattgg

SEQ ID NO: 1043 - DNA, 23 bp, Homo sapiens
gagtccgagcagaagaagaaggg

SEQ ID NO: 1044 - DNA, 23 bp, Homo sapiens
gcgccaccggttgatgtgatggg

SEQ ID NO: 1045 - DNA, 23 bp, Homo sapiens
ggggcacagatgagaaactcagg

SEQ ID NO: 1046 - DNA, 23 bp, Homo sapiens
gtacaaacggcagaagctggagg

SEQ ID NO: 1047 - DNA, 23 bp, Homo sapiens
ggcagaagctggaggaggaaggg

SEQ ID NO: 1048 - DNA, 23 bp, Homo sapiens
ggagcccttcttcttctgctcgg

SEQ ID NO: 1049 - DNA, 23 bp, Homo sapiens
gggcaaccacaaacccacgaggg

SEQ ID NO: 1050 - DNA, 23 bp, Homo sapiens
gctcccatcacatcaaccggtgg

SEQ ID NO: 1051 - DNA, 23 bp, Homo sapiens
gtggcgcattgccacgaagcagg

SEQ ID NO: 1052 - DNA, 23 bp, Homo sapiens
ggcagagtgctgcttgctgctgg

SEQ ID NO: 1053 - DNA, 23 bp, Homo sapiens
gcccctgcgtgggcccaagctgg

SEQ ID NO: 1054 - DNA, 23 bp, Homo sapiens
gagtggccagagtccagcttggg

SEQ ID NO: 1055 - DNA, 23 bp, Homo sapiens
ggcctccccaaagcctggccagg

SEQ ID NO: 1056 - RNA, 20 nt, Artificial Sequence
  source: /note="Description of Artificial Sequence: Synthetic oligonucleotide"
gacaucgauguccuccccau

SEQ ID NO: 1057 - DNA, 23 bp, Artificial Sequence
  source: /note="Description of Artificial Sequence: Synthetic oligonucleotide"
  source: /note="Description of Combined DNA/RNA Molecule: Synthetic oligonucleotide"
gacaucgauguccuccccautgg

SEQ ID NO: 1058 - DNA, 23 bp, Artificial Sequence
  source: /note="Description of Artificial Sequence: Synthetic oligonucleotide"
  source: /note="Description of Combined DNA/RNA Molecule: Synthetic oligonucleotide"
gacaucgauagccuccccactgg

SEQ ID NO: 1059 - RNA, 23 nt, Artificial Sequence
  source: /note="Description of Artificial Sequence: Synthetic oligonucleotide"
gacaccgaugucaucuccaucag

SEQ ID NO: 1060 - RNA, 23 nt, Artificial Sequence
  source: /note="Description of Artificial Sequence: Synthetic oligonucleotide"
gacaugaaugaccuccccaucag

SEQ ID NO: 1061 - RNA, 23 nt, Artificial Sequence
  source: /note="Description of Artificial Sequence: Synthetic oligonucleotide"
gaaaucaagguccuccccauagg

SEQ ID NO: 1062 - RNA, 23 nt, Artificial Sequence
  source: /note="Description of Artificial Sequence: Synthetic oligonucleotide"
cacauagguguccuccccauagg

SEQ ID NO: 1063 - RNA, 20 nt, Artificial Sequence
  source: /note="Description of Artificial Sequence: Synthetic oligonucleotide"
gcgccaccgguugaugugau

SEQ ID NO: 1064 - DNA, 23 bp, Artificial Sequence
  source: /note="Description of Artificial Sequence: Synthetic oligonucleotide"
  source: /note="Description of Combined DNA/RNA Molecule: Synthetic oligonucleotide"
gcgccaccgguugaugugautgg

SEQ ID NO: 1065 - DNA, 23 bp, Artificial Sequence
  source: /note="Description of Artificial Sequence: Synthetic oligonucleotide"
  source: /note="Description of Combined DNA/RNA Molecule: Synthetic oligonucleotide"
gggccatggguugaugugacgag

SEQ ID NO: 1066 - DNA, 27 bp, Artificial Sequence
  source: /note="Description of Artificial Sequence: Synthetic oligonucleotide"
gcccgggtggaactggtagccatgaat

SEQ ID NO: 1067 - DNA, 26 bp, Artificial Sequence
  source: /note="Description of Artificial Sequence: Synthetic oligonucleotide"
gttgaagatgaagcccagagcggagt

SEQ ID NO: 1068 - DNA, 27 bp, Artificial Sequence
  source: /note="Description of Artificial Sequence: Synthetic oligonucleotide"
gcttccgacgaggtggccatcaaggat

SEQ ID NO: 1069 - DNA, 27 bp, Artificial Sequence
  source: /note="Description of Artificial Sequence: Synthetic oligonucleotide"
gcaccatctctccgtggtaccccgggt

SEQ ID NO: 1070 - DNA, 26 bp, Artificial Sequence
  source: /note="Description of Artificial Sequence: Synthetic oligonucleotide"
ggtggaactggtagccatgaatgaga

SEQ ID NO: 1071 - DNA, 27 bp, Artificial Sequence
  source: /note="Description of Artificial Sequence: Synthetic oligonucleotide"
gccatgaatgagaccgacccaaagagc

SEQ ID NO: 1072 - DNA, 27 bp, Artificial Sequence
  source: /note="Description of Artificial Sequence: Synthetic oligonucleotide"
gcatcctcgtgggcacttccgacgagg

SEQ ID NO: 1073 - DNA, 27 bp, Artificial Sequence
  source: /note="Description of Artificial Sequence: Synthetic oligonucleotide"
gcagagcggagtgctgttctcccaagt

SEQ ID NO: 1074 - DNA, 26 bp, Artificial Sequence
  source: /note="Description of Artificial Sequence: Synthetic oligonucleotide"
ggtcggtctcattcatggctaccagt

SEQ ID NO: 1075 - DNA, 26 bp, Artificial Sequence
  source: /note="Description of Artificial Sequence: Synthetic oligonucleotide"
gcaataaaaggtgctattgctatagt

SEQ ID NO: 1076 - DNA, 20 bp, Sus scrofa
gggagtctttcgctagggtg